European Patent Specification EP 3 265 098 B1, published March 26, 2025. Title: COMPOSITIONS FOR MODULATING MECP2 EXPRESSION. Applicant: Ionis Pharamceuticals, Inc. The sequence listing filed with the application follows.

SEQUENCE LISTING (328 sequences)

SEQ ID NO: 1 - DNA, 80001 bp, Homo sapiens
gctaccatcaactctttctcctagactgttccagggccttgcaactagccttgtgctgtagttttgtttcatcacgtccagttctccactctacacctgcaacatagatcagacagctcctggctcaaaatcctctgagggcttctcatcttagaataaactctcggttctggccgggtgcggtggcttacgcctgtagtcccagcactttgggagtccgaggcgggcggatcacttgaactcaggagtttgagaccagcctgggcaacatggtgaactcccatctctatcaaaaatacaaaaacttagccaggcgtggtggttcgcatctgtggtcccagctacttaggacgctgaggagggaggatcgcttgagctcagggtggacgttgcagtgagccaagattgcgccactgcactgcagcctgggtgacagaatgagaccccatccccaccccccccaaaaaagaatgaactcccagttctcatagtggccccagctgcctttccaatcacattccctaccactctccagcaacactgacttcctcgttagtccccaacatgccaggcatagtctctcctcatgtcctttgaacttgcctggaatgttctttccccagatattcatatgagggagtaaaatgagggtgaaaaccagcagatatctaaatagcacccccttcacttagtttatctttctcaaagcccttatcactatgtgaaatgatatattatacttatttgtatgctagtatgaatcttcccggcaagaatgttagtttgctgtctgttcagtaccgtgcatccagagcctggaagagtgcctggcacatagcaggtagtcaataaatgaatgggggcaagcagccaaatcagaatcaggttttcttgctaagcatagaactaacagaaggatcattgaatggattggataatgactggcatcagggtaaggtccccttaacaaacactcctgtcctgaacacctggttagctaacagttttctcatactcttattttcccaaaacacaattgctggatctcagctccaaatcaactcttctaggaaagtgaaaaattgctggatctcagctcccaaatcatatcttccaggcagagctaacattgccccttattcacacctccaccaaaccatctgatccaacagtgacaggtgtcacgaggccttggcatgcactctcttcccccgccagagttctgcgaaagccagggttgcgatttgttgtcagtttattccccgcctctatgagagtgtgagcactgggcaggctcggatgaaataatgcattgagtaggcctctgaaaccaaggcccctcagctggggcaacgtcaggctccagggtgggcaactttgctgcttctgccgaagatagtgatattgagaaaatgtgggtgcaatgaaacgcttattgcagcgcactcggtgcatctgtggacagagggtcaatcgcccctcagagcagcgcaaacaggcgtcccaagcctaggccttcacttgccccagcatccgcaagggtccattaatccttaacattcaaattccgcccactaaaccagtccctccgcgcccaagccgcctcttttccccaaacgacggccgaaagcagccaatcaacagctggaggggtccgcccccttttccctggccgaaatggacaggaaatctcgccaattgacggcatcgccgctgagacctcccccctcccccgtcctccccgtcccagcccggccatcacagccaatgacgggcgggctcgcagcggcgccgagggcggggcgcgggcgcgcaggtgcagcagcgcgcgggccggccaagagggcggggcgcgacgtcggccgtgcggggtcccggcgtcggcggcgcgcgcgctccctcctctcggagagagggctgtggtaaaagccgtccggaaaatggccgccgccgccgccgccgcgccgagcggaggaggaggaggaggcgaggaggagagactgtgagtgggaccgccgtggccgcgggcggggacccttgccggggggcgggggtcaggggcgggacgtggcgcgggaggggcccgcggggtcggacgacacggctggcggatggcgtccctcctctctaccctccccctcccgccgccgccggtggcgactctcccctcggcccgtcacccgtgctcgcgggtgaccgtcctcggcgcggcctccctggagccgccttcgcctgacgcccctcttcctcccgccctcgacgcgcatcccggcccccggccccgcgggcgcccctgtcgccggggttcgcctgtcggggctgcgcgcgctcctgcccttctcggggctttgggccgcggcgccgtcgcgcgcccgcggccccggcctctccctggatcgcgctctccccctccctccctcgcgcgccccctctcccgttactcggcccccccaccggcgcgcgtgcgcacttcgcctcccgtcgggagagtgcgccacaagggctcctgagctctcacccccatctctgggctttgcctccccctccttctcgcccattccatgaatttctgccccccgctacccccccgcgagcgagtaggtccaccggctcctttccccatctagcaggaacaagtaggtggggattattatccacaaaagggactagacattgtgttctgggtcccacaactcatcataaagaggtggttatagttcccatcaggagccgtgggtaggggactgtgcgtccagcagcacccgaggctcttcggcgccagaggctctaaggtgcgagcgtgtccccagggtgctcagaggttctttggagtgctgtggcctcggaatgtgagcaccctcccatcctaccctccccttcgccggcgatcttccagttacataagtggagtgggacatagtaggtaacgggctctcatcgccctggagcgctcgggatcaccggtaccagatggggcaagttcatcgcgacgctgtggctcctgttaattgtgcctgaaaggttatcctctgttcagtttggtcatgaccgaatcacccaaactgaaactcagatgacttttatatggcagtggcaatgtttctgtggttttgcactaaagacttaaggtcattatgaagagtgtaaaaggattgctgtcgcaggggagaccgtttatgacattgctaagtatggaccccgagggggaaaaagctcattctggaattgctctgtggcggttgcttctgttgcgagtgtgttcgggtgtgggttggtcacagcagaaatgggctccaccacaaaattgatattcctgactcatggtcaggcagatgtgtgcttctggttatttttccaggaacaggaatgggctctgccgagcctttcacacgttgtgtctctgctgtgcgggatcagtaccccagactgtgagataacaggatcgaattcaggggttggttggtgatccaggaaccatacctacttggatgtgatactgagtggcctagacgttgtaggactctcataagttttagacattttgttatactgtaaaaatgaagcatatacggcctcagtagtaacattgcactaataggtaattattactctagagaattttgggttccatggctggaatgttcatcagtatctcagcaatttcagttaataaccagattaagctgacctcttgagtcttttgaaatctgctgggtccctataataagacagggtctggattttttaatcttttgggaatttccaccaaggatttagggaaataggcttttatgggcttttcaggatttctatttcaaatcccaatgaggaagtctaggaaacacttgcttttattttcttgcctgaatatgtcagaaccttaaatcacccaatcaatctagaagtactacagttgattaaagtaagtcaccacaggtcacccattcgtggcaggtcagctaggtggctgatcactggaatacagtcatatccccaggcatacacacgagcctcacttgacgatcccaaagtttgtacatctgagcttgagacgtgacaagttgaggtctctgctttgttcttcatagttggcagtttgtctcctcgggtgcccctccggttagctgtttatcatacgtctagccctatcaacagtgcaggcagcttccagagtatagttttctctgcaaagtgcctggtggaggggtacctccttttccattgtcctaatggctccactgggcttccataccagccctttccagtgtcttaacagctcaaagaaacccatctgtggctttcttgttagcactggcctatcacaccttcctattgcctgttaactaaaattttgcctggaatgctttaagcttagagtactgggtctttgtttcacccgattgataggagagtgtcatgcagtcagccgaactccgacttctgtgctgtttaaatccttaggtaggtctggggcaaggcacaaaccactgtgtattcaaagggttatggtgcttgcattctgtgtgtatatgtttgtaatttccaaccagagtcgtttcccgtgcctgccctgcctctgtgcaatctagtctagtagggtagggaggcaagctgtggagtttgaaaaaaaaaaaaaaagctagatgagtttaataggctgttaccccctccagaacattcctcccatgtggagatgaaacgagaagttcatttctttaacctaaaataaagaacaacagagataaaattgttagttccttattggagcctggtttccattgctaatgtacctgcttgggactctgcatgataaatgacgtgtcctggaacctgaaatcttttataaaggttaatatcagcagaaatcttttaattagctaagagcagcttgttctcaagctgcccgagttatcttggaggagagaatcacaggaaatgtttgatatttctagtaaccagtgttttcagtgcgtggggtaaagcacactcctagactggccagtcccaaagagtgtggcaggacacctgcttgttttccctgccctctgctatggtgacatccttgcagaccagtcttgcgtggctggcagacgcaatctttttttcttgggtagagcattatcaccgctgcgatggaaggaccttgtcctcggtgcctccataccagccctttccagtgaaactactgctgtcccggcaagcccctgtgcgtgtgcatcattccgggtaggacaagatgtgaacaggtccctcttctttgggcttaagtagaagttgtgctcttctgcttttacctgtgtgctcttctgcttttacctgttctcttctgcctttctcttgcaagaaacctgtcgaaagcttgctttgcatgccattgcttaaatactttgatggtatgtatggtatgtgggataactgagtgggagccggaattggggggtgggcagggcatccccacccccacccccacatcaaagggggaatgaccatttcgttagagaataaagcctgagtcttataacttcttcaagcacatgtatgctgggtctcctggcgtgtgaatgtgttcccgctgtgctgtgtggctgttttgcagttactgtagacactgtagtctgggctctcattattgcctctgaagttgacaggaccaagccttagtaaggatgcacttgtcttcctagcccaagagctaggggtgttttatatatatattaactttcttttttagatttcataaactgctctcattttctcttttctttctttctttttttttttttttttttgagacagtctcactctgtcacccatgctggagtgcagtggcacgatctcagctcactgcaacctctgcctcccgggctcaagcagttctctgcctcagcctcccaagtagctgggattacaggcacctgccaccacgcctggctaatttttgtattttttttttttttttttttttttttttagtcgagacggggtttcaccatcttggccacgctggtcttgaactcctgacctcgtgatccacccgcttcagcctcccaaagtgcagggattacaggcgtgagccaccgcacccagcctctggctcttttctttttgacatgaaatcttaagttaattatcttaaactttaagaactagaaggattcttagtccagcaccatcagtttacaaacaaaaaaaacttgtgtccctgagaagttgtgacttttccagggcctcctagccaggataccagtttggtttttattatatagctagccgagtaatactattaacttgacttctgggatttcaaagtattctatgacttgactgtttaagggaattatgaggcctcactgaacctcaaaagataattttaggtaccatcctggtagctgtagagcagcaacagaccagtaaaagacttggttggtgttgcccttcttctgggtttgattacatgagtaattgtgtgaatagtctctaagttgtatgctctgagctttcgtttttagcttataaaagtgctactcttgggccagcatagtatcagaaattagctaattcatatggggcagtttaggctttaactaggaaatgatggttatcttaatgacaaaaaaggtactgacaaaagtccttttttgaacatgtgttcaaaagaaaaagagaaactatcaaactaataactgagtttgttgaacatcgagattgactgatctgagaggcttaaaactgattgccctgaaatagacttgcatgttttggatgatggctttgggtctcccagagcacttggtttcccttggtgctgattttttctctcaggattaaagcccctttatgtgatgttgttacagcagcttattgcaacttcattcagctgcttgaaaaagaagggagactgcctctaggttccatgtgttctttcagggatggtattttgatgttgcgtattctcttgaacatgtattcttccctgagaatttctgtgtgccgtggtagaagaaatacttgccagaaatcgccactcatggtatgcttttgtagtgtcgaagtgtcccctagaggtgacaaggcttgtgatagtgttgattctaacaagcatgaatctttcctttattttagcactgtgtgttacgtgccagtaatttgcagcttatcctttgtttctagctaggtaagctgggaaatagcctagtactttgtctatgtgtttatcttcaaaatgtcccaaatagccctgggaaaaaggtcgtgcagctcaatgggggctttcaacttacaattttctttgttttaggctccataaaaatacagactcaccagttcctgctttgatgtgacatgtgactccccagaatacaccttgcttctgtagaccagctccaacaggattccatggtagctgggatgttagggctcaggtaagtaaccttcctttttttttttttagtatatgtcctggtttggccatctgttttttttttttttaaaaaaaaaaaaaaaaggaaaagaggaaaaaaatatactactcttggacagtataaaagtaccccaaagactaaagacataactgtgccaaactgtgccatataataaaaaaaagtcacttccctgagccctgaaaggtcagtgtgtgtagggttacttggtcgccacagcgtgatctgggggcgggcgtcagattagagccggaactggtgatctgcaacttcagttcaccttgaagcaggtcagctgagctgagagcgcttgcactgagcccttttgcgctgctgctgttgccttagcggtcttcagcatgtgtttgctttggtttggggtaaatggcttagtggtcaacattagtgagcagtggtaatgcattttcagatatgggaactggtatgtggttggttccctagaaggacaccctcctgaaagctgtctcagaacaccgggggccatggctaatgtcatgtgcttgctacactcctcccatggtaactaaagagagtacccagatatacatctggttcttgggactctagaggaggatgagtactttgtaaaaacctgggggccccagtcattctaggtctgacactcaggtgctgtatcagctgcagtttgaactacttggcaccattgtgtggactttagttttgtaaaaatgaatggttccttaatttctcaaccttcaggctcaacatctcaagctgtttgttgttgttgttgttgttgttgttttgttttgtctttttgattagtggtcactccgcatttgatgttttgacatgtggatttcagaacttctgtgtggtaaagcagaatgttccaattgaattttcccattttttttcccctaagcaaaaatgtgagttttcacttatgcggccattgtgattccgactgagaccctaagtcgttctttgttgtctctctagtggtttctgacacctcagtgtgaagctgttgtagacatccataagaaatagcctgcttagggattatgtgagggcaaggtttggctgaaggagaatagaaggtgtggaaggaagcggaagaccagaagagcatcacactgcctcaagtcccaaatttgattctgctcctgatcctgtgactcaaattgtcattctcttttactgctgtggggtgtgctctgggcccagctgacaggacattctttgtactccacgtatttatgctggtgggagttgtatggctagtgctttgtgctttgtctcagaaattgtgtggactaaatgtaatatgggcagtgaatgggtttcttctggaagatgttaggcctggagggtggtttgggtttttacgagtctttttctcagattacagattacgaatggatgttataaaacaggcagtgttgacaccatacagtttctcctaagaaatgtacagagagttcaacctgaggaagctaattgaaaataaacttttaaaaagaaatgtagaaagaggaaatttaaaaagtatcttatgaatgggaaagatgtagccatttgagcttcaaagaacttttgagggaattctcaaaggacagtacccgtctttagtagataaatgcttgatatctatttttcttcttttactttttaaagaattactaaaataatacatggatttatagaaaaatcaaaccacttaaaaattgatcaggtggctgggcaaggtggctcatgcctgtaatcacagcgctttgggaggcctaggcgggtggatcacctgaagtcaggagttcgagaccagcctggctaacacggcgaaaccccatctctattaaaaatacaaaaattagctggccatggtggcttgagcgtgtagtcccagctactcggaaggctgaggcaggagaatcacttgaacctgggaggcggaggttgcagtgagccaagatcacaccactgcactcctgcctgggtgacagagtgagactcggtctcaaaaaaaaaaaaaaaaaaaagtatcaggtaaaaaaatgaaagctccccgcttaatctctgctcccactacccagaataactgctgttaatagcttaatgtagatccttctaagtcttctaagactaaactgtgtactttttgtgttgtaattaacaggagggtttttgttttgttttgttttttctttttttgagatggagtcttgctctgtcatccaggctggagtacagtggcacaatcttggctcactgcaacctccacctcctgggttcaagtgattctcctgcctcagcctcctgagtagctgggattacaggcgcctgccaccacacccagctaatttttgtatttttagtagagatgggtttcaccatgttggccaggctggtgtcgaactcctgacctcaggcgatccacctgccttggcctcccaaagtgctgggattacaggcgtgagccaccgtgcctggcctcaggatggtgttatatatacatattctgcatttttccatctcatatattcatctctgcctcatttcttttaaatagcagtgtagtccagggctgacttaccgtcatgcatttcgttgtctctctatgttattaaaaatgctacaggattgaaattcctcatgtgccagtcattttgaagaatggctgcctagacttggaatttctggtggataccaccacatcactgtccaaaatggctatcccagttcccacaacagtctgagaaagtgccattttcccatatcgtcccagaattggatatacatcttttaaattggtgccgcttggattattactgaggctaaacctcaataatcattgtcatagctcttaatgtattaaagatgttaactctttgtcatgcagatattttcctgttttgtcttacgtcttgattcttgtctttctgatatataaaatttatgttatgatttattcttttgctttcatacttaggaaatccttttttactctttttttttttttttttttttttttttgagacggagtctcgctctgtcgcccaggttggagtgcaatggcgtgatcttggctcactgcaagctccatctcccgggttcattccattctcctgcctcagcctcccgagtagctgggactacaggcgcccgccaccacgcctggctaatttttttgtatttttagtagagacagggtttcaccatgttagccaggctggtctcgatctcctgaccttgtgatccgcccgtctctgcctcccaaagtgctgggattacaggcgtgagccaccgcgccccgccaggaaatcctttcctactcttaacaacagatcaatagtcatctatattttcttcctaaaaaacctgatgatgtattatattcatacatacgtatttaatacatacaaaagggccagatgcggtggctcatgcctgtaatcccagcactttgggaggctgaggcgggtggatcacctgaggtcaagagttcaagaccagcctggccaagatggtgaaatcccgtctctactaaaaatacaaaaattagccaggcgtggtggcgggcacctgtaatctcaactactggggtgactgaggcaggagaatcgcttgaacccaggaggcagaagtttcggtgagccaagatcacgccactgcactcctgcctgggcgatagagtgaggctctgtctcaaaaataaaaaataaaaataataattttatagttaagttgccctgtgtttttcctgtgattaaaaaaaaaaatacctgttttgtatttaactttggggtgggataaggtatagcccacttagtcagttgtgtctaagccacttgatgaaccagtcaatccagtcttcacctttaacaaatgctgatttcttcaagtgagcaaaatatctcttaaactttttcctattttctctataaagttgcttttttctgaattttttctttatgaggcttgatgggcagccctatcagcagacaatcattcattcacccaacaaatatttgagtatctgcttcaagccaggggcagtgctaagccctggaagtggtatcttctccttatccgggagtggggctacagtgttcattccagaagactcaagaaaatagcagatcatcacaaaagtaggttttacataaatgaggaggaatccacagggttgtgtatatgtgtgtgtattttaaattctgacataagttggagctttagggtagactgtgacataagagtagtttgttttccaactcatgtaattgccggctgatttttgtcttgaattatgataatggtaacttctgttgaaacaattctgtattcatcttagcttggttgggatgcaataaaagttttgtactggtaaaaatgataattttcttccatgatgattttgaagcttttctgtaacacctgataaaaatagaggggccaggcatggtggctcatgcctgtagtcccagctactcgggaggatgaggtgagaggatcccatgagcccaggagttttaggctacagtgagccatcatcacaccactgtactcctgtactctagcctgggcagcctcgttctttagagtaagacactgtctctttaaaaaaaaaaaaaaagaaaaaagaaaaaaagaaaaggcttttagtgaatatatttttagggtagcaagtgtaatttttataaattgcattatttgaatctaataaataccctcaaagctgaagtcgaattctgattttgattgaaaatattttttacttaaaggaagagggatagaataaatgacacgattaaggaaaagacttcttgtataaggccggggttttttaaatgattttttgaatagttagatggacaatacggaattaaaaaggtggtgtaaaaagttatacggggctgggcacagtgactcacgcctgcaatcccagtactttgggaggccgaggtgggtggatcacctgaggtcaggagttcgagaccagcctagccaacatgacgaaacatcatttctactaaaaatacaaaaattagctgggcttggtggtatgcacctgtaatccagctactcgggaggctgaggcagaagaatcgtttgaacccaggaggcagaggttgcagtgagccaagatcgtgccattgcactccagcctgggcgacagagtgagactccatctcagaaaaataataatagaaaaaagttatatggggctgggcatggtggctcatgcctgtaatcccagcagtttgggaggctgaggcagcttgatcacttgaggtcaggaattcgagactagcctggccaacatggtgaaactccgtctccactaaaaatacaaaaattagccaagcgtggtggtgcgtgcctgtagtcccagctacttgggaagctgaggcaggagaatcgcctgaacctgggaggcagaggttgcagtgagccaagatcatgccgttgcactccagcctggacgacaagagcggaactccgtctcaaaaaaaaaaaaaaaagagttatattgtaaagtatctctgctaccctgccccaaacattcatttctttccctggaggcagccactattacctgtttctttaaaaaaaaaaaaaaattgtggccgggcacggtggctcacgcctgtaatcctagcactttgggaggtggaggtgggtggatcatgaggtcaagagatcgagaccatcttggccaacatggtaaaaccccatctctactaaaaatacaaaaaattagccgggcatggtggcgggcacctgtagtcccagctactcgggaggctgaggcaggagaatcgcttgaacctgggaggcagaggttgcagtgaactgagatcacgccgctgcactccagcctggcaacagaatgagactccatctcaaaaaaaaaagcgtgtgtgtacccgtgtgttaaatttttattataaaatatatataacaggctgggcgtggtggctcacgcctgtaatcccagcactttgggaggccgaggcaggctgatcacgaggtcaggagatcgagaccatcctggcgagcacggtgaaacctcgtctttactaaaaatacaaaaaattagccgggcatggtggcgggcgcctgtagtcccagctactctgagagcctgaggcaggagaatggcgtgaacccaggaggcggagcttgcagtgagccgagatcgcgtcactgcactccagcctgggcgacagaccgagactccgtctcaaaaaatatatatcgatatatataacaatttacagttttaatcatcttaactgtacagttcagtggcactgagtacattcacattgttgtacagccattactaccatccatctctacaacctttcgtcttgcaaaactgaaatttcatacctattaaacactaactcccacttctcccctttcccccaccccaccctctggcaactactattctactctttgtctctattggacatatttttgtgtgtttaggtttgtgtatatattttacatgtgtgtataaatacacaagggtatgtgggcgttgtgtttttacacatactataaaatattgtgcacatttgtttattttaatgtatcctgtagattatttagaatcggttcatacagagccgtatcattccttttaagggttgggtttaaatagtctgttatggatgtaccacaatttatttaaccagtttttaaattttttacttattttttttaatgtttttttagagacaggatcccactccatcacccagactggagtgcaacagcatgatcatagcttactgcagccttgaactccggggctgatgtgatcctcccacctcaggctctcttgtagctgggactacagggatgtgccgccatgcctggctaaattttttatttttatttttatttttatttttggtagacacggggtttcactgtgttgcccaggctggtcttgaactccttgggcttgagtaatcctcctgccttggcctcccaaagtgccgagattacaaccatgagccatggagcccgacaagagtagccttttatttgcagaccattagagaaaaagttgcgtgtaagtagataagcatacgaatttatcactgcaatactgtttgtagagatcacagagctgttaggctaggaagaagtttttagcagttagcactagaaagcaaaactttggaaacttccatttcatcaaaagtgacctcatctgagtagggcatgtgagggaaggacctttttactcgacaaggggaacttgccagttcttgtttgtgaaccttgaagaaagtggagcatttttattttgggaccattctaggttgtggtagttccttggtactcggggttggagaatctccctctgctgctggaccttctgcctcctcatgctgtaatatgcataagaggtgtcctagaagtattcaggaacaggctgtggttgctttgttgttctgtgactgttgaactctttatatagcagtacttttttaagctgtactaattgagcatttattatgtgtcagttactgtgctagctgctggaaactatcctaccctcagcagtcttctggtctaatgggaggtacagacaggcaaatgggctatgactttacaagaggctaacttctgtgatggagagaagttccagccactaagggagcacataaaaatcagaggagatcctaccaagaattgggaggtaggtcagggaggagacttctttgaaaaatggcatctaagacctgaacagcaaggaaacattagctaggtcaaggacaaagcatcagtggggagagatgcatgagtcttttggaaggaccagcatgtgtagaggctctgacaggagagaatctctcaggcccattcagagagtccactgtgtgaagacgaggcatgaacaaccagccaggacatgtggagaggagcatttttctttttttcttttttctttcttttttttttttttttttttttgagacgtctttctctgtcacccaggctggagtgcaatggcatgatctcggctcactgcaacccccacttccagggttcaagcaattcttctgccttagcctcccaagcagctaggattacaggcacccgccaccatgcccggttaatttttgtatttttagtagagacggagtttcaccatgttggcctcaaactcctgaccttaggtgatccacccgtctcggcctcccagagtgctgggattacaggtgagagcccccacgcccggccaggctcggctttctttccaggccccgtcacactcttagatgttccctgggccccagaaggcagcgtgaggtgctctgcccatctatgctgtccttttccaccccaccctatccactgggcccctggggctcccactccactccaggtctcttcatggacccttctttcccttcacttctgtcccaggagacctgggagactcatgggaacaggcatcatcttctccagcacagttcattgtctaatgcacgaaagtgctgggctgtgagaaggtcaggagcttacatggaatgggagtcagctgtggtacaaagtacgctgcttagttctactgattttttattttttatttttacataagactttgatggtaaaggaagcagtgtgtgagcaagctgactcctgtcttgtcaagtaccaggtccactctgatgagcccctgtggacagcactgctgtaactccccaagcctgggctcaggaggtgggccctaagcgctgttcccagctcttcctccatgctgtcagctcttccaccattcttcctggcgtcattctaaggtcctgtcttcccccgccctcttccttcctggcttctacgctcagctcaagtagtagctgtttgggtacttttcacccagacttaggaaatgttatcagttggtcgtattcctgtcagccctcttactatggaactcaaataggacagattcagctgaattcccagccctgtggttgcactctttgtctgccctgcttccccaaggtagcctgctccctaaaggtcaccgagatactccccatgcaaggtttttgttgtattacacatgacaacatggaataaagtgttttgcaaatttactggatgatatcctactatgtggaacatcctacaacttactcttttcactcaacatttgacttttgaacctggtctgtattgctccgtgcagaccaatgttcattcatttgatatgtctccttgtgccatagaaatagttttacaatagaagcctgtccagagccatgagggagaaggggattgtagagaaacaaggattggcatctggtttatgtttacatcctttagtcctgttaaccgagaagaagatatttttatttccatgtttgcgaaagctttccacaaaaaaaagcatccattttctagacttattaatagggcagtccaaaggttttatttttagatttgaaagaaagcaaagtaggcttctgagatatgcacatttccctgtgtccctgtctcttttgcaacattccacattgctgctaaaacttgaacatgagcactttcaagcatgtgcttactttctatgtatgactcattttttaaaacattaaagcattttcggccgggtgtggtggctcacgcctatattcctagcactttagaaggccgaggcgggtagatcacttgaggtcaggagttcaagaccagcctagccaatatagtgaaaccccatctccactaaaaatacaaaaattagccgggcatggtggcgggcgcctgtaatcccagctactcgggaggctgaggcaggagaattgcttgaacccaggaggtggaggttgcagtgagcagagatcgagccactgcactctagcctaggtgacagagcgagactctgtctcaaaaaaataaaaataaagcattaaagcactttgtctggtggtatgtaagttttggcattacttagataagttgtattttaagtctttctacacacaataacttatttttaaaatacaagtttctgtgtacttccgggttttgtgtttttgtaaacagcagaaggtattagtccatattaagtactaatttgttctaatattttcagctgtttttggaattacacttggcaaaaaaatagacaaatgtctgcagttgtgacagtttgtttttttgttctttttaactccagaataaataattctagtgagtttttttcttggcttgtaagaacatgggaatgattagagtcatcataacacttaagtagttatagaaggttgaacatctgtagtcagttgtataaaatttcctagtcatccttccaggttgtttaagacaaacaaatacatagtatttattaagctcttataaattttaattgtaaaacatcattgtacaaaactttgaaaatgcgtataggtacaaagataaaaaattaggccaggcatgccatggctcacgcctgtaatcccagcactttgggaggccaaggtgggaggatcttttgagcccaggagttcaagaccagcctgagcaacatattgagaccctatctctacaaaaatatcataaaacaaaatagaatcactctggcgattccactatccaaaaaaaaaaaaaactgctgttaatatttggtatgtatctttctagaccaaggcctccaactttggttgagaattcagccgggtctgtgaccttggatgggaaaaacattcactctttattttcactaatgtctctgaaaacccagatttttagctgggcatggtggctcgtgcctgtaatcccagtgctttggaagcccgtggagggcagatcacttgagcccaggagtttgagaccagcctgggcaacatagcaagaccctgtcttttaaaaaaaaaaaaaatccagccgggtgtggtggctcatgcctgtaatcccagcactttgagaggctgaggcaggcagatcacctgaggtcaggagtttgagaccagcctgaccaacatggtgaaatcctgtctctactaaaaatacaaaaatcagccgggcatggtggtgggcgcctgtaatcccagctactccggaggctgaggcaggagaatcacttgaacccggaaggtagaggttgcagtgagccaagatcacaccattgcactccagcctgggcgacagagcgagactctgtctcaaaaaaaaaaaaaaaaatccacattttcttcaatgacaattgtaagcaacagatcatggtagtattagaatagcagtgactgtcaccagtagagatcaaagatactttcatatcatattatagttgttacagatattttgaaatatatatgtccatcactgcttcaaacttaaggtaattattagacccatctctagatctggttatttaatgatttactgaagaagcacatattatttgagaacgaactcttgaaatatgttgttaatttctgtgcattttacacatttcaaaacattcttctgaggaggggtccagaaggccaaaagggtccatggcagaaaaaggttaagaacacctgttctgtactttgtaccatgtggctacaaatataaaaacagacgttaagccgggtatggtgatgcacacctgtagttccacctacttgggaggctgaggtgggaaaatcacttgagcccaggagtttgaggccagcctgggcaacagagcaagaccccatctcttaaaaaccagtcagcacttgactagtcagttagtgggggaaaacacaggtacagtaaaaggagtcaaaattacacttaaacttaggtcatcttattatatcaaacatttattaacatgtttagtgttttgtgtatattatgcaaagtgtaatgcaactaaaactgtttaacacttctcgatatcacataaatttgttggtgcataatagcctaaaagttacttttgctgttggcattttattttattacttacttatttatttatttatttatttattttgagacagagtcacactgtcgccaggctggagtgcagtggtgcgatctcagctcactgcaacctctgcctccctggttcaagcgattctcccgcctcagcctcctgactagctgggactacaggtgcgcgccaccatgcccagctaatttttgtatttttagtagagatagggtttcgccatgttggccaggatggtcttcatctcttgaccttgtgatctgcccacctcggcctcccaaagtgctaggattacaggcatgagccaccacgctgggcctgctgttggcattttaaacatccttctagagtctttcttatttgcctgtaagcacgtacacatgttgttgttgttttgagacaaggtctgtcgcccaagctggagcacagtggtgcaatcacagctcactacagcttcgacctcttgggtgcaagtgatcctcccaatcagcctcccaagtaggtgggactacaggtgtccgctaccatgcccagctaatttttgtattttttttgtagagacggagtttcaccatgttgcccagactggtctcaaactcctttgctcaaacgatccttccgcctcggcctcccaaagtgccgggattacaagtgtgcacctctgtgcctggcccacatattgttttagatgaatgagatcatatatgtacttttgtaacttgctacctttcctcaacaaaatgttgtaaatatccatgtccataaaaatagacgtatatcttcacttttccctaaaatgaaaataacttaacttgcattttcttttttgtttttgtttttgttttgagacaggctcttgctctgttgctcaggctggagtgcagtgatgtcacagctcactacagcctccacctccagtttcaagtattccacctacctcagcctccaagatagctaagactacaggcacatgtcacgacgcctggctaatttttaaaatattttttgcagaaatgggatttcactatgttgcccaggctggcctcaaactgctggcctcaagtgatcttcctgccttggcctcccaaagtgctgggattacagtcgtgagccactgtgcccagcctgcattttcttattataaaagtaatacatgttcaatggacaaaaaattttcagaaaatatgcaaagatgaaaagtaaaaattgtccataaatctgtcatctacagataaagataacttctggataatgtttttctaccatcatttttagtaatcacataacatttcgttgtatgtctatgccttcatttaattaagaggcatttccattatttctgcatgttcatgactctgaatgatgatatgtctgcctgctgatggctacaaccctgtttctgcatttcaaacctctctcttgagctccagatttgatggcctcgtcagcatttacttgagttgctcataagtgtctcaaatttaacaagtcccagtcttgatttttttcccccttcaaacctattcctcatgttgtctctatttcagtaaacaatatcaacatccacccagttactcagtccaaaattctaggagtcatccttgattctgctctttctttttttttttttttttgagacggagtctcgctctgtcgcccaggccggactgcggactgcagtggcgcgatctcggctcactgcaagctccgcttcccgggttcacgccattctcctgcctcagcctcccgagtagctgggactacaggcgcccgccaccgcgcccggctaattttttgtatttttagtagagacggggtttcaccttgttagccaggatggtctcgatctcctgacctcatgatccacccgcctcggcctcccaaagtgctgggattacaggcgtgagccaccgcgcccggcctcttttttttttttgatacggagtctcattctcgtcatccaggctggagtgcagtggtgcaatcttggctcactgcaacctccgcctcccgggttcaagcaattcttctgccccaacctcctgagtagctgggcctggctaattttttgtatttttagtagagatggggtttcaccatgttggccaggctggtcctgaactcctgaccttgtgatccgcccacctcagcctcccaaagtgctgggattacaggcgtgagccactgcacccgccctgattctgctctttctctcatcatccctgatctgtcagcaagtcctgttaggccaaccacttctcagcatctgcactgccagtatgctagtccaagccacaaaacacctctcagaggtacgcaacaggactttgttgttgttgtgtgtgtgtgtgttttttttttttttacggtagaattattttataacttgaagtgtagggatgaccttccttttaaaattttatttattttcttaattttttattcccatagattttaggggaacaggtggtatttggtgacatgagtaagttctttaatggtgatttctgagattttggtgcacccatcacccgagcagtgtacactgaacccaatttgtagtcttttatccctcaccccctcccaccctttccctcaagtccccaaagtccattgtatcattctgatgcctttgcatcctcatagcttagctcccacttatgagtgagaacatacggtgtttggttttccattcctgagttacttcacttagaataatagtctctagttccatccaggttgctgtgaatgccattaagtcattcctttttatggctgagtagtattcctttgtatatatatgccacaatttctctattcactttctgattgatgggcatttgggctggttctatatttttgtaattgtgaattgtgctgctataagcatgcgtgtgcaagtatcattatgcaacgggacttcggatgacatattgaacaacttcctcactgatatccttgtgaaacgctacatatttcatgggtctgtttgttataccaacactcaattctgaatgatggaattatttcacatttagtctctttttcatctagccattatagtttagtttaaacaccaagttccattcctgctgcatgctgaaggatttgcagtacatcaggctatagtccatcaattcattccacaattgagtaagtaaggtatctatagtacctcaggccctgtgttaggcagggatggggtaacctagacagatttggtacctgtcctcatggagcttgactttagcggcagagacagatcttagataattgtaccagtacttaagtgttcagaaggacaagtatggaggtgggagccactccagtcctctacagtcacgtgctgcacaacaacgtttcaaccgacaacagagcacacatacagtggtgttcccataagattagaatgccatatttttactgtaccttttctatgtttagatatacaaatacttaccattgtgttccagtgatctacagtattcagtatagtaccatgctgtacagttttatagcccaggagcaataggctatataccgtatagcctaggtgtgtagtatgctacaccatctagatttgtgtaagaacactctctgatgttagcacaaataaatcgcccaatgacacatttctcagaacatatccctgttgttgagcgactcatgactgtacaatgggggaacagctcagcctgccttccccaaggaggcaacgccgatgcagggaaccgagggttgaacagaagtgggcaaggtgcagagaggaaaaaggctttccagatggagaagagcatgtgtgaaggccctcagtctggcaagagcttagtcctgtgtggcaggagctgaacgaggggttaggggagagtggcaaagggtccgggccatcagagaggtcaacaggggctggatcatgcaggattttgaatgttaacatcagagcgatagaaaacatgaagggtaaggtggtttgggttttgaatttttatcaaaatattgcaactactcggcaacaagttagatataacaaaagaggtcatcgtaaaaacagcagtctaccccttccccttcccttccctgactcagacatgacagcttttaactgtttctgattttagttcctttgatggttacctccaaaattaaatcatatgcttatacatctttcttgatttgccaactttagggaactgtgttaactccctgaaatgaaagagaatgacttagcttacgttacctccccatgttgaaattcatattcacatttctctgtaattttttttttgagatggagtctcactctgtcgcccaggctggagtgcagtgatgtgatctcggctcactgaaacctctgcctcccgggttcaagcaattctcgtgcctcagcctcctgagtagctgggactacaggcgcacaccagtgcactgggctaatttttgtatttttagtagaggcggggtttcaccatgttggccaggctggtcttaaactcctgacctcaggtgatctgcctgccttggcctcccaaagtgctgggattacaggtgtgagctaccatgccaagcccacatttctctgtaaattttaaacagtattttagtccatatgtcagttcccctctttttaagataaggatattaataaccctacttttccttccactttccctccttaacttctgcgtcttaaaagctgtacttgaccatacccattcttgcatttgttaacatgtgtgttctgccctgcaaccacagccaagttgtagcttaattctaaagtcgaaaataacattatttacattattacacatgtgagtattgttcttggcgagaccaaataatgaatgtgcccaggattacatttccttctttacagatctggaccactcaaaggagaatgaccaatcaaggtcaaatggattcccttttcttagactctgtcacctgcttaaaatccttgctaggatttaatctacttcatattcaaaccttggcttgcttatatagctctttgttttgcccaccatttctagttgcctttttattttgtttactattcctccttgattatgttgtaaaatgctattagcagtgctgtttatttcgtacgattcggctttttccccactgaagacctttctcttggaaggcctctgcccttctgcaatctgggcaagtatctgctctttgatttaaggttgcatatacagctgtacctggaccttctcctcactgggctcttgggttggagcccgtgtcttaaaacccatatcttcctttcacatggtttactccctcgttttctggactgcatccttaaataatgtgctcagatagagtgcatggggagtaaactgtagtggataccgttgtcacctaccccatatccatttcttctttgcccattcctaacagaatcctgatattattcacctttctaccttattcccaacttcagaaaggatccttaagtcattccacacattgcattcctttggcaactgttactggtcaaggatggacatacgatctaagttggttcactcagactgaagggaaggacttccatggcacgttcagggaagactttctctttttctctcactggagtaagtgagaaaggtgttgctgggggctcttctgtaacctcagactgagggacaaagcctgaggataaagcctgctcaccaaggaaggcggagcagagaaacgggaagaacctgggtcttgatgccgttgcttagctggtgattgcactgtggctggggcctgtcctacctgagctagggactcagataggatggactttcttactgaatgagccagcttcagttttcttttctgttacttgtaaccaaaagcattgtaacagataggtcttctgagtcactgcatgcctgaaatacctttcttctactcttacacttgattggctgagtatagggttccaagttgaaaatcattttttctcctaactttggaggcatctcttctagtatgcagagtaacaaatgcaacaaatgcctgatgccaatcttattatggttcttttgtaggtgcccttcttttctcttccttccctggaagtttttaggatttcgtctccttatttttagtgtcctgaaatctcatgagaatatgtctagagttgtgtcttgttcactcgttgtactgtggtcattcaatctgaatacttttgtcaactcttttttttaaaaaaaaattactaatttacatgctttcattttctctatggggactactgtttaactttggacctcttatattggtcttctgtcttctctcatatttttcatttattgggcggtggggggtgctctgaattttggaagatctcctgcatttattttctttttccttttttctttttttttgaggcagagtcttgctctgtcacccaggctggagtgcagtagcctgatctcggctcactgcaacctctgccttccaggttcaagcaattctgcctctgcctcccacgtagctgggattacagacctgcaccaccacgcccggctaatttttgtatttttaatagagatggggtttcaccatgttgccaggctggtctcgaactcctgacctcaagtgatccgcccgcctcagcctcccaaagtggtgtgagccaccgcacccagcctcctgactttattttctatcccttctgttaaattctttatttcagccaaacctttttttttttttttttaacttactgtgaagcctgtgtgcctactgcctagattagacaattgttaacattttggcgtattttcctggtctgtatagatagggtgcatttttatacctttttgctcaccatttaaaaggaactcacagatgtcacgacatttcacccctaagtacttcagtatacatctcctaaaaataaggacattttccaatataagcacaataccccgatcacatctttaaaagttaacaataattctctaatgttatcaggcacccactttaaattcagatttcctccaaatgtctcttatcgctgttgaggggctccaaagcaattaagatttatacattgcatttgaatatgcttcctttgtctcttatttatttatttattttattttgagacagagtctcgctgtctcccaggctggagtgcagtggtgtgatctcagctcactgcaacctccgccttccaggttcaagcgattctcctgcctcagcctcccaaatagctgggattacaggtacgcaccaccacgcccagctaacttttttgtatttttagtagagacagggtttctactaaaccatgttggccaggctggttttgaactcctgacctcaagtgatctgcccgcctcggcctcccaaagttctaggattataggcgtgagccaccatgcccagcccctttgtctcttttaacaagaacagcctacccacctctccttcacttgtgatactgactttttgaagcagtcagcccaattgtcatctagaagggcccacattttaagatacatatttttagagatggcgtgtcactatgttgcctaggctggccttgaactcctggcctcaagtaatcctcctgcctcagcctcccaggtagctgggactacaggcttgtgccaccacgactagctggcccacattttagatgtctctcttttcttgtgatataatttaacttgtttgtccatatatattacttgtagacaagaagttaggtctacaggcatgttcaggttaaacattttgggcaagaatatttcataggcagtactgtgtacttcatatagcatcagctcaccaggcacttaatggttggttaccctgtggtttgtgatgctacgttttaacacttgattaaagaaggaggtgactgccaaatctccccattgtagacatacagttttcctgtggtaattgatatataatctgtgatgtgatgctttggcaccatacaaatatcctattgcccaacagccatttgcataattattttagcattcattgatccttgcctgaaaccattattacattgggggttgcaaaatgatagtttttttaattgtcacctcttctacatttagtactgtcattcctctgtaatgaattttccctcatcaaataaggaggcattatatttcctcctaaaaagacagtatagatgcttaatctttgcctttattacatttcagagtaaggagttggtagaataatcacctcaaatggtggcaaaatatttgctgttgtgtttccttttctctttcatgtcaatatggactcatagggatttatttattaaatgttttacaattcaaattgggtcaacaagagtcccttcatgttggttcctatattctcctggcataccctcattaattagtctttgagcaatttcttgttttctggcacaagatattccatcccaatatgtgcttttcgtgtcctagaactgattccaaggagctctggttccttatagtggcaacggtatttagaatccaacatgtgggtactaaatgtgctgattcttactggggtaacattatatctaggcactttcagaggacatcgctagaaaatatattcagtttttattttttatttttaatttttttgtagagacaaggtctcactatgttgcccaagctggtttcgaactgagctcaagcgatcctcccacctcagcctcccaaagtgctgggattacatctgtcagggcaaactgctggtaaatattttcacaaaagaaaaataaaaaaaccaaagtgctgggattacagatgtgagccactgtgccctccattttttttttaagtcataaatacataatgatgtcttctatggcaatttaacattacagggttcttccttaacttttttttttttttttcttttttttgaggcagggtcttgctctattgcccaggctggagtggtgcagtggtacaatcctaattcactgcagcttcaaatgcctaggcttcaaacaatcctcctccctcagcctcccgagtagctaagactacaggtgcatatcaccatgcccagctaatttttaaaaattttttgtagagatggggggtctcgttgcgttgcccaggctggtctcgaactcctggcctcaagtgatcctcccatctcgatttcccaaagtgctgggattacaggtgtgagccaccatgcctggccaacttttatttgatctgtatatatcttttccttacactgaaaatgttgggtcttactaatgttaacatagttacttatttgctttatcttgtaatagacataaaattacaaaattataataccaatattacgataaatagctgggcatggcggcgctcgcctgtagtcccagctactcaggaagctgaggtggagggactgcttgaacctaagagtttgaagctgcagtgagctgtggttgtgccactgtactcctacccggacaacagagtgagtggggggaaaaaaaagaaataatggaagatccagagaaagccccaaatatttaaaaattaaacaatacactttgcagcttcctcacctctctcagccttcatagaattgaagagagttagggccttgcactagattaggctttgccttaaggaaatgttgtgtttgatttgatcttttatccagaccattaaaacttccttaacgtttattagtaataaggctatttcactttcatatcatttgtgtgttcactggagtagcacttttagtttccttcaagaactttgattcacaacttggctaactttggtacaagaggcctagcttttggcttctcggctttcaacatgcctctcactaagcctgatcatttggtttttggtttaaagagaaagacatatgactcttccttttacttgaatgcttagaggccattgtagggttattaattggcctaatttcagtactgtcttgtccaagggaatagggaggcccaaggagagagagagagatgggggaacagctgattggtggagtagtcagaatatacacatttatcacttaagttttgccatcttttctttttctttttcttttttttttttgagacagtcttgctctgtcacccaggctggcatgcagtggcatgatctcagttcactgcaacctctgcctcctgggctcaagcaattctcctgcctcaacctcccgagtagctggtattacaagcgtgcgccaccatacccagctaatttttatattttttagtagagacagggtttgccatgttggccaggctggtctcgaattcctgacctcaagtgatccacccgccttggcctcccaaagtgcggggattacaggcgtaagccactgccgcctggccaagtttgccaccttttttattttttttattttttgagatggagtctcactccatcacccaggctggagtgcagtgatgcaatctcggctcactgcagtctctgcctcctggattcaagcgattctcctgcctcagcctcccgagtagctgggactacaggcatgtgccagcacgcccagcttgttttttgtatttttagtagagacggggtttcaccatgttggccaggctggtctccaactcctgacctcaggtgatctgcccggctcagcctcccaaagtgctgggattacaggcgtgagccaccccgcccggccaagtttgccatcttttatgggtgcagtttgtggtgccgcaaaatgatgatagtagtaacatcagagagcattgatcacagatcaccataacaaatataataatgagaaatttgaaacattgtgaaaattaccaaaatgtgacagagacatgaagtaagcacatgctattggaaaaatggcactggtaaacttgcttgatgcagggttgccacacaccttcaatttgttaaaaactcagtatctgcgaagtacagtaaagcaaagcacaatcaaatgaggtgcgcctgcatattacaaccaagaggcttttcgcagaaacacgagtgtgcttcaacattcaaaaatcagttggtgtaattcaccacattaagataataaaggaggccgggtgcggtggctcacacctgtaatcccagcactttcagaagccgaggtggacagatcacttgaggccaggagtttgagagcagcctggccaacatagtgaaatcctgtctctactaaaaatagaaaaattagccgggcagggtggcacgcacctttagtcccagctattcgggaggctgaggcaggtgaatccttgaaaccaagaggcggaggttgcagtaagctgagatcacgccaatgcattctagcctgggcaacagtgagacccagtatccaaaaaaaaaaaaaaaaaaaaaaaagataataaaggagaaaaaccatatagtctattcaataaatacagaaaacgcatctgacaaaattcagtgccctttcatgataaaaattcagcagattagaaatagaggaagtgcatgtatgaaagagctacagatagattgtacttaattgtgaaatattgaacatgttaccccgaaaatcaggaaaaaggcaaagatgtccactctaaccacttctattcaacattatactagaggtcatagccagtataatgaggcaagaaaaaacataagaggcattaatatttaaaggaagtaaaactgtttctatttgtaggtaatgtcgaaaatgtgaaagaaactatcagaacctgctagaactaaaaagtgaattcagcaaggtctcagggtacgagatcattcaaaaactaatcagaaatgaaatttcaaatgcaatatcgttaggaataatttaataagaaatgtacaagatttacacgctgaaactgaaaatgttgctgaaagaaattaaagacctaaataaatggaatgttgtaccatgttcatcagctgaaagactaagtgtctttacagtgtcagttctcccttcattgaactgtagattcataaccccagtcataactgcagggttttttttgtagaaattgattgtaaaatgtatatggaagctgggcacggtggcttatgcctgtaaaccagcactttgggaggctgaggcagacagatgacttgaggtcaggaatttgagaccagcctggctaacatgacgaaaccccgtctctacaaaaaatacaaaaattagccagacatggtggcacacacctgtaatcccagctacttgggaggctgaggcatgagaatcacttgaacccggaggtggaggttgcagtgagccaagatcatgccactgcacgcccgcctgggcaacagagtgagactttgcctcaaataaataaataaataaaacgtatatggaaatgcaaaggacctagaacatccaaagtaaacttgaaagagaacaaaattaaggggcttatgtgatgtgactttatagtcatttgatttttaacagaggcaccagaacagtccggtgcgggaaaggaaagtcttttagcacgtgccggatgatggcaaatgacatccataccagacaaaaatgaaccttgaccttaccctaaatattagtttcttagagttgccacaaactaggtggcttaaaaccacagaaatttggctgggtgcggtggctgacgcctgtaatcccggcctttgggaggccgagtcgggcagatcacctgaggtcaggagtgcaagactagcctggccaacgtggtgaaactttgtctctactaaaaatacaaaaaacttagtcaggtgtagtggtgcacacatataatcccagctagccaggaggctgaggcaggagaattgcatgaacctgggaggttgcactgagccaagattgcaccactgcactccagcctgggtgacagagtgagactccgtctcaaaacaaaaccacagaaatttgctgtctcataattccagagtctagaagtccaaaatcaactgtcatcagggccatggtctctgtgaaacctgtaggggagtccttccttgcctcttcctagcttccagtggttggcaacctttggcattctttgatttgcagctgcattacttcaatatctgtcttcctcatcacacagcattctccatgtatgtctctgtctttacatggcctccttcttgtaagaacaacagtaatattggattggggcctgccctactccagtgtgacctcaccttaactaattacacctgcaacaacgctgtttccaactaaggtctcagtgtgaggtactgagggttaggacttcaacatatcttttttgggggacatagtccaacccatgacactacttcacaccatacataaaaattaattcatgagagattatagacctaaatgttttaaaagctaaaaatataaagcttctgcaagaaaacataggagaatatctgtgcagtccaaagaataaggttttttttaaacacaatttcactctgttgcccaggctggagtgcagtggtgcgatctcagctcactgcaacctctgcctcccgagttcaagcgattcccatgcctcagccttccaagtagctgggattacaggtgtgcgccaccatgcctggctaatttttgtatttttagtagaggcagggttttgccatgttggccaggctggtctcaaactcctgacctcaagtgatctgcctgcctcggcctcccaaagtgctgggattacaggtatgagccaccgtgccaggccaaaaaaagatttattaggatacatgaagcaatagctattaaaagaaaaaataaattggacttcattaaaatttaaaacttttggtcctcaaaagataccattaagaaaatgaaaagacagagctgggcgtggtgaggcttgcctgtagtcactactgggtacttgagaggctgaggcaggaggatcacttgagcccaggagttctaggccaacataggcaatatagtgagacagtgtctcttaaaaaaaaaaagaaaaagaaaaaacaaaagaaaataggctgagagctgtggctcatgcttgtaatcccagcactttgggagtacaaggcagatggattgcttgagctcaggagttcaagaccagcctgggcaacagtgaaatcccatctctacaaaagatacaaaaaattagccaaccatggtggcgtgcacccgtagtccatagtcccagctactcgggaagcagaggcaggaggattgcttgatcccaaggaggtcaaggctgcagtgagctgaggtcgcgccaccgcaccccagcctgggtgactgagtgagaccctgtctcaaagaaaatgaaaagacaagtccaccaagaaaacagttgagaccagtcatagaaaaaatagaaagtcatatctgacaaaggatttgtattcagaagaattcctataactcggtaataaaaagacaacctgatttttaaagggtgaaaatattttaatggatacttttttttttttttttgagacagagtctcactgtgtcacctaggctggagtgcagtggtgccatcatacatagctcactgcagactcgaactcctgggctcaagtggtcttcctgcctcagcctcctgcgtagctaggactacaagcacgtgccactatgcctggctaatttttaaattttttgtagacatgggctggtgtgtgtctgtgttgtctaggctggtcttgaactcctgggctcaagtgatcctcccacctctgccccccaaagtgctgggccaccacgcctggtgtggtgtcaccagagatgagccaccatgccctgcctgatacttttcttttatcatctgtttatttcttgtttatgggtgtttctgttctgattttatgactattctgtattctaagatttctctgagaatattatttgtttcctctaaggacagacttggtctctcttccatggggctggttcttgagccgccagggatggggggaggacctgggtagctgctgcgctgccccttctctgctgtggtggagtggcccgttgcctgcggggtctgtctctgaagggtggtttggagaagttctgtggaggcgaggcaggggtcagctcttgccccatggaccctcagagactgggaaaaggtaggcatcacctgggctgctgccagccacatcaagagcctttggggtgggtggggtgggggccggggaagggaaggttctagctgttgatttagaaaagacccattgatttcttgcctgagggaagaagtggcaccttgccactccaagtttgctctgctcaccagccccaacagcatcagcctcacctgggagcttattgaaggtgccctgccccaaagcttgtgggtcgggatctggcagtcagcagcccccaggtgttgcacacatgacagcactgcttgcccctcctctcgtctggtctggtctggtctggtctggtctggtctgagagcttctttggggctctgacaggtatacaggctctcatctgctctacagctctcttgtagtacattcctctctgttccattagtcaacatgttcttgcctacttccagcatctagaaatttgctgagtgtatcttatccgttcagaggtcctctcctgctattgcctctgttagaaatttcttccctttcatatgtctgtacttcggtttctttgaggtttgaagggtcaagtggcaattacatgtaggcagttggccatcctctggtgaaggctttaaagcccaggaataacaagatccattatgtctaaaactagcaaaaaccctacctgtcacatggtgaactgaattagaggtgatggggacagaagccagattggagtgagtggaaggtgagggagtggagattgggtatagacaactctctttaagaagttttgttgtgatggtgaccagaaaaataggagtggggtagagggggatgagggtgtttttcacgtgggtgaatatgagagcatgtttacatccttctgggaatggcccaggagagaggggagcgtgagaaggaggaaatggggacctggaggagcagactccttgtgtggaggggggaagcggcatctagagctgttgcaggaggtgggctttgagtaaatgcttcctctttggtaaagacggggaacgggaacggtagaagttgcacggaccctttgttaaagctcagaagctgagcgagaattagagcttaagtttatggagtagtcagaataaagtacccctaactgtattcttgcacagtgcaggaagccaggggtctgaaatcaagatgttgcagggctccattccccccagagcctctagcatggatccttccttgcctcttccagcttttggtggctgcctggcagtcctagactttccttggcttgcagttgcattgctccattctctgcttgtgtcttcacatggccttctctgtgtccccgtattcttctctggatgcttgtcactgtattaggcccaccctaaatccaggatgatctcatatcaagatccttcacttaattacagaagcaaagaccttccaaataaggtcagagccacagggtctgggggttaagacatacacctaactattcggggctaccatcgaacccctgtagaagcctgtccatttccaggatagcagagcccaaggaagggccagaagtccccccaaaacagttgtttgcattcaccagattctaagctataagcagatgggcagtggcagtcggtcctaatccatataccattggcaacaatagtttagttcactgtagacataatgagatgcttatcttctgctaagtagtcctcatggtaacagccatattactcctggctttgagtgacagcgctgtgctcttgtctggtgcccatatacttcagcagctggaaacaagacagtgctcatgattcaccggaaagtttctgtagttaaaatcaagtgatcccttgagtctattctaatatttgtctgtaccatgttctgtgacgagacatggaaacaaaacattaagaagtgaaagtatctttgattatgctcttgaagacaactttttgtttgtttgttttgtttgagacggagtttcactcttgttgcccaggctggagtgcaatggtgtgatctcggctcactgcaacctccgcattcccgggttcaagcgattctcctgcctcagcctcccaagtagccaggattacaggcatgcaccaccacgcctggctaattttttttattttagtagagacggggtttcaccatgctagtcagactggtctcaaactcctgacctcaggtgatccgcctgcctctgcctcccaaagtgccgggattacaggtgtgagccaccgtgcctggccgaagacaactttttaaagatgcatatgctctgggctgggtgtggtggctcacacctgtaatcccagcactttgggaggccaaggcgggcagatcacctgaggtcaggggttcaagaccagcctggccaacatggtgaaacaccgtctctactaaaagtataaaaattagccgggtgtggtggcgggtgcctgtaatcacagctactcaggaggctgaggcaggagaatcgcttgaaccccagaggcggaggttgcagtgaattgagactgtgccactgcactccagcctgggcgacagagtgagacttggtctcaataaataaaataaaataaagatgcatatatgctctgaaggctggctacattttattttttctcaaacaacttttacagtggatagtgctgtaaaagttgtttagctctggtcattttatcttttttgtgatctgcaaaaggagatccttttccttttcactgcctctaatacccaactccaatactcctttgacctcacaggcacttagaatccatcagtggctccatcttttctcagacttcacctccttcgtatccttattcctctcctttgtagcttcagtgccagtcagacgtcgttactccctggcacactacctcagcccttcggcactttcttgctttgttatattcagtcgacaaagccccagcctcatgaaattcagtcatgtctgccccatgcctgctccgtcctgaagctgaatgtgactccttcattgattccccctttaagttcatgtctaccccaggtaaacttcttgccgccaagcccacctgcatactgcagttccccggtctctcctagcccctcccaccctcctcatcagctgtcacacctccttgcagctgatatcttagttcccagagagcacagaagcaagctcaagagagtgtctacaggccagcgtctactccttcgctctgcctccctcatgctgtcacggagcgcctgtcccaggccctcactcctgttctaaggcatctctccagtcctctactgcactctcccccatcagagattcctccctcgcctgccctagaaacttgttgctacttctcccaccttgacaaaagctgctcccaaccccccacctgtctagcatctctgttttcctttaccagcaagactccagtccctgtctccacaccctcttcaaccttctccagttgttcctttgctgccacagctctgccaagctgctccatgaggtctccagtgatgaccttcatgttgttaaatctgggagctgcttgtcacttcttttcccagagctgtcgtcgtcagttaaccccaatacccatacgagacaatcctttccctcccttgagtctctgcactgatgtgcaccttctcagtgcaaaccacagcttttgtctctttctagctgaatacatgactgactgtgcttatcttagctgtcacccctgctggagcagaagctccacaggacaggattgtctccttgattcacagatgtagctcaagctcctagaacagtgcctggtgtctgtgggtcctcaggaagtcctaggtgagtgtgtgaatgtctgtcctcctcggtcttttctgtttcgcatgtgatgttggaaggcctcaggttcaggcttttcttctccaccctcactcccgaagtgattccgtccagcctcatggctcccaaatttatgtctccaggctgactgggtcacgggaactccttatcctccctagaccttctctttccctggtcttctcctttccagtaaacagcaactccaactcctgctcctcaggccagaaacctggcgctggttacctcatttgttcacaaatactgttactccacctgcaagatggatacaaaatctcatgagttcccctgcctccatggcccccaccctggtccaggtgtccagcttccctgcctctgcccttgccccctggttctttgtttagtcctgcaatattgtgctcttctgttcagaaccctccagtgggtccctgcttgctcagagtcacagcccaacaggatcacctctcttgccactctcccaccactcatgcactgcggcctcactggcctcctggctcctccctggaccctccaagtatgcccctgcctcaaggccttgacctctcctctgccctctgtcccaggtatcacacatgtctgctcaagtgtcaccttcccaatgtggccttccccgagcacacccatgtctgtaagtcaggcagcctgcctctgccccaccagttccccctgcctagcataggacttgtcaccatctgccacaagctgtgttactgcttggttttgtttgtgctctcccactcccttcccctccctccctctccccacccctatagaatctgagtcccatgaggacagagatttttttttttgcctcttcctcaatatatccccagtgcctagaatcatgcatattttaatttattgagtgaattaacaaataaattctgcagtgggacattgctctaaggttttgtcttataagagggacagaagaacatgcagcctgctctgctgttggctccttagcttctccatggctaacaggaacaatattgtttatgagataatcaaagccatagtcatgagttagaaggtacatataaaggcaaatatgtggagattgagttactttggcgggggcggaggggtgtgtagttatctgaaaacatggaacaaatcaatgagagtctaaatagcacccacatatttgcccctcttttaaaacatacctcctttatgagtgtagaatttaacagcacagtttcccagtgcagctttgcgaaacaagagaaatgaattttaaaggctgtcaggtgcctttgcaatctgtggcttagtatttgtgtaacaacatttgtgttttgccaacagatgtactgcttaaagtacccatgagaatggcctctgtggttttctactttctcggatggaaccttaggaactgattattgagaagaggctgatactgcccacctcagctcccaggcaggcttcagggccttggttactactcctttgggccctcactgacccttgcagacgtcttttgcaacctctgtagccagaagagacaactgctttctggcatgttgctctttccctaatggctttatgagcttcttgaacaccaaagcatgtgtgacttcctcacgccttcccctgtatagtatagcacccctaactgtatgtgtaaggagaaggagtgagcaattgatggcgtccccctggatctccaagggaatgggaaggggcagggtttctggattcagtcatgtggaatctggtcgttggtgtctaaatgtgcctgttacttgtgcccaatgtccaggttcaccaggaggcttagcctgctcatttccctgctagtagctatattttgggagagcattttttatgctctaattgaactttgtgggtctcagcaatttgaacaatgttttgtttttcttctggtcaggttacaaaggaaagaaaaggaatctggtgttgtaggaggtggtgtgttgtgtaattacttgttttttttttttaagtttttttatatttttgcaacaaggcaagttttctttgaataaataatgctgggagcttatcacatagaaggcatatgtgttgtactcagtacattctgaattatctgggtttatttttatctcttgaattcacttataaacaattcaaaggctgcttttttagctaacagaaataggaagagaatctcagaatctgttttgtcattttttcaatgggttgagttatagtgattatgctaactcggtggaaaagcagtgtagtgagtaaaccccacatacggcatatcatgaacattttgttgcttttttggcttctgaccatcttcatacctttttttgtgttaaaagtctccccattgtgtatatcttagtaagaggcaggtggaccctagtttctacctaagaaaacctgaagatggggttgggggcctgtggtgtacttccttctcatgctgtccatgaccactgcagtggctttgtaaggatccaggacccagggcccctcagtgggtgtcttccatttctcaagattgcctcttggttgtgagatgacggttgctgctctagtcattgcatccactcctccaggtaggaagaaagaggtcataggggaaaggcaaaatggcacttgacatcttaacttctaggcccattcaatatttccatttccatcttcacacccatcatcttgtcctagggaacaaacagcaccagcagctcagtagctataacagcaattattatttctcacacatgggtctgggtcagctgcaagatgggattcagatctgttctcaagcctgtcgttccaggacccaggagggagaagcagctgccaggggaagtctcttcgtaggcggaggtcaggagtccaagaggagtgagcagagtcacagaagcctcttaaagcctcttcttcccccatcccatcaacacgtgagcaagcccagagtcagtgggtgggaggtgtgctccgcccatagtcagtagaacaagagcaagcttgaaagagaacgatgaacaggagtgcactcggccactgtctccttagccataacgtagtcccatggtctgctgggaagcggggaataactctccttagctgagcgcagggtctcattagtaaggcagatggagaacatggatgttgggggacaactggcagtgcctgccacaggggaatggatatattccctccccttgctctctggaaactaggggatggcgatgaagcctaggtttggccaaacccattctgccttcagggactttgactcttgagggacagtgagggattagtcatggtggtggcagttgagtcacaaaaccagcagtggtggctaatgtccagtgatgacatgcaacagtgcccagggtgggtgtcccaaccagcaggtccctgcagtataaccttggctgtgtttgcagtggtgcagcctctattcctgctgcttttctgagcctagttctctagttctctctccatttccagatctgctgcccaagaactcctttgtgattgaatttaaccagagttgatttctgttgcttgaaactcaggaccttgatgcagtgtgcagggtctgggcaaggtaaaaacacactttcatgatttcgcctcaagtatagtagatgagcttaggctttttgagccaggtagccttgggattaattctcagctcttgcacctagcaggtgacctcagcaatcaagtcacttgccctccttgagcctcagtgttgccctcagttaaacattgctctcgtgtgttgctgagcattcagtgagattgtatataaagtgatcattgtgaaggtattgggacataatttgggaaagcgtcctggtctaagcttttgattggctctccatcatttgggtaatgggatagtgatttaggagtatcatagcagctcaaggggcccttctggaaagggtatgaggaaggtcagggacaagtctgaaatgaatcatcctaggcttaatgcctgtgactgggcagtgggtacaattatctcaggctagtcagtagtcatttattgtgagaatacatgggcagattttttaatttccttctcagtctagacttgaatgcaaacagttcttattgctaacttaccactagtcaccactaatgaacaaagactatgaacaggaaattcataaaagaagagatacagatggccaatgaagataggaaaagagttctgcctgctggtaatcaaagagatgcaaacgagaacaaaaatgatgccttttcacctaccaaatttgtcaagattaaaaagaaagcaaagagccagcgtcagctgatgttcatacctgcacctgctcggtagcttgctaatgttctgcctgctccacacgccaggccagcctccacggcgcagccaggtgaggcctttccttgtatacaggcacgtttggattcactgttgcataagtgagacatgtgcatgcttcacaattcaggaagtgcaaactccagagtgatgcaaggtctgagtgtccctgctgccctggtctcccagctgcctaggcctctcttcagggaacggctgcatccagggtcttgtctgtgtcttttgaggtgttctatgtacacgcagacacatctaaacctatttttattttccctgcacctgcttgggctactgtaagctgttaaatttttttttctaggaatttgtccattttgtctgactagcataaagttgttcatgttatagtttatacatttgcaacatctgtaattatgtctgctttttcattcctagtgtttgttgtttacttgtaccttctcccgtttttccttgtcttggtaaaagctcattaggttcattggtcttacaagaagcagacatgtaggcattattgccctgtattactctgtgtctcttttctagttcattaaattctgcttttgcttttatctttattattttttctatggtcttagagtacattctctgtgttttgttgttgttgttgttgttgtttgttttttgttttgagagagagagtcttgctctgtcgcccaggctggagtgcagtagtgcaatctcagctcactgcaacctccacctcctgggttcaagtgattctcgtgcctcaacctcccgagtagctgagatttacaggcatttgccccacacccggcaaattttttgtatttttagtagagatggggttttggcatgttgaccaggcgggtctcgaactgctgacgccaggtgctccacccgccttggcctcccaaagtgctgggattacaggcatgagccaccacgcctggccctaacttcttaagttataaatttggttcattgatttttctacccttttttcaaatgtaaacatttaaggctaaccctctggaactacttcaactgtatctagcaagttctgatagtattgtcactttaagttagcccaaagatattttaaattttctttgtttcttcctttgactcacatattattttaaaatgtgtttttcaatttccaagcacatggctttgggtttgttttttttttttcctagttgctctagaaaaaaaaattgactgcatgaggtggctcatgcctgtaatcccagcactttgggaggccgaggcgggcagatcacctgaggtcaggagttcgagaccagcctggccaacatgccaaaacctcgtctctactaaaaatacaaaattagccgggcatggtggcacacacctgtagttccagctactcgggaggctgaggcaggagaatcacttgaaccgggaggcagtggtcacagtgagccaagattgtgccagtgtactccagcctgggcaacaagagcaatactccgtctcaaaaaaaaaaaagaaaaaaagaaaaaatcaacttctaactaaatggcactgtgatcaaagaacttggtctgtgtgacaccagttcttgcagttggttgagaagtgctccatgacacattatccacaaccagtggacagaatatgtcaccaccaagcatgggtgcaggattctacatatattcattacctctgtcttatccgtttgttgtgaaagtattttctcttcttactgtcattttgtttacttgatttatcaactgatggaatacgtgttaaaacctactgtggtgatggacacatcagtttctccacagagtttggtcattttcattttattatttattttgaggccacattttcagttttagatacagtttcacattcctggtgtattgaaccctttggtattatgaagcgaccatactaatatgttatttttttttaaattattatttattttatttatttttctttcttttttttttttttgagacagggtctccctctgtcacccagtctggagtgcagtggtgcaatctcagctcactgcaacctccgcctcctgggctcaagtggtcctcccacctcagcctcctgagtagctgggattacaggcttgcaccagcgcgcctggctaagtttttgtatttttagtagagacagggttttgccatgttgcccagactggtctcaaactcctgggctcaagcagttcaccagccttggcctctaaaagtgttgggattacaggtgtgagccaccacgcccggccatcccagttttttattttcctcctttctgtgtctttatgcatcagtgaggtggagcttttgaaaatgtcagatagctagattttttttttttgagacggagttttgctcttgttgcccaggctggagtgcaatggcgtgatctcggctcactgcaacctccacctcccaggttcaaaacaattctcctgccgcagcctcctgagtagctgggactacaggcacgtgccaccacacccggctaattttgtatttttagtagagatgtggtttcaccatgttggccaggctggtctcaaactcctcacctcagctgatcacccgcctcagcctcccaaagtgttggaattacagacgtgagccaccatgcccagctgatagctagattttttttttttttttttttttgagacggagtcttgctctgtcgcccaggctggagtgcggtggcgcgatctcggctcactgcaagctccgccccccgggttcatgccattctcctgcttcagcctccagagtagctgggactacaggtgcccgccaccacgcgtggctgattttttttttttttttttttttgtatttttagtagagacggggtttcaccgtgtcagccaggatggtctcgatctcctgacctcgtgatccgcccgcctcagcctcccaaagtgctgggattacaggcgtgagccaccgcacccggcctcgagattttttaaaaaatccattgtctgtttcgtcctttaacatctatttgatttctgatgtatttagattcatttatagcatatttgtgcattctatttttccatattttctgttcttttaaattttccttctcctttcttgccttctcttagacttttaaaaaaattgtagtaaaatacacatcacctaaaatttaccatttttaaatgtacagttcagtggcattaaatacaaattggaggccaggcatggtggctcatgcctggaatcccagcactttgagaggctgaggtgggaggattgcttgaacctggaggtcgaggttgcagtgaggtgtgatcacactactgctatagcccaggcaacagagtgagaacctatctaaaaaaacaaacaaacaaacaaacaaacagattggcatcacacagtgtgtgtgctgctgtgctgtgctgttatcatttaacattaaaacataaacatcagcactgttatggactgaatgtttgtgtcccccaaaattccagtgttgaagctcaaacctccaatgtgatgttatttggagatggggtatttgagaggtggttaggtttagatgaaatcaggagggagggtgggtttcgcatgatgagattagtgtccttataacaagagacagcagagagcttgctttctccaccatgtgagtatgcaatgagaaggcagccatctccaagtcagaaagagagccctcaccaggggctgaatgtgctgacaccttgatcttggacttctagcctccagaactgtgagaaatttcagttgaataggccccccagtctgtactattttgttatagcttgagcagactaatacacccatgttatgaaaagctataaacatccctttaaaggccacctaacgcgtcgtattacctcatgcatcttctctgctgagctttccaaaagagtggcttaggctgggcctggtggctcatgcctgtaatcccagcactttgggaggccaaggcaggtggatcacctgaggtcaggagttcaagaccagcctgaccaacatggagaaatcccgtccctactaaaaatacaaaattagctgggcgtggtggcgcatgcctgtaatcccagctacttgggaggctgagccaggagaatcacttgaacctgggagatggagggtgcagtgagccgagatcgtgccattgcattccagcccggccaacaagagcgaaactccatctcaaaaaaaaagagtggctggccgggcgcagtggctcacgcctgtaatccccgcactgtgggaggccgaggtgggtggatcacgaggtcaggagttcaaaaccagcctggccgagatggtgaaaccccgtctctactaaaaatagaaaaactagccaggcgcagtggcaggcgcctgtaatcccagctacttgggtggctgaggcaggagaatcgcttgaacctggggggcggaggttgcagtgagccaagatggtgccactgcactccagcctgggtgacacagtgagaccccgtctcaaaaaaaaaaaaaaaaaaaaaaaaagtggcgtatgttcccggtctccacctctcattcgccagcccctgtgaccaaacccctgggattagatctccatcgggtccctcccctcaccctaacctcacatgcagtggttcctgagaagctgctgtttatctgatcacgggatccagcaggatctgagggctcattcactgaatctgtactacccaacaaggcaggcttgtccttacccacacttttcaggtgaaaacttaatcagattcaagcgtttatcttagtggcctcttcgtggtgtgtgatttccttcttgcagctctttactggctaaaactcttcactgggagttaaaccaggtgtggtccttgaccctcatcattttgtcccatctcctatgctgggctctgtatccttgtctccaagcagtctcgtgtgacagggaagttacctattattgtatggtcccctcttcttgtcacctctggtgtggcacttgttccatttcttgttcaatgaatgtgatttgtgaatgtgccacatctgtgggaggaaggcagttcgcagcaagagttgtagttcccttgctttgccctgagggccaggactttacactagatttttttgttgcattcctgcactcataaagtacacgtaaacttagaggtggtgtgttaaatgctagaacttaaaactgagttcagctaggctcaagtgccccacaatttttgtcccaccagacaatttcatgaatatctacagattgttccctcaatatgcctcaatattgaggcatattgatttggggagcacagacaagtcaaggttgatgtgcatccgctgaacatgatcttaagttgttgaagtaggtattattaatgaacgaacgtctattttagctccaagagcccctggtcttccagaagagactcccaatgatcttccagaagcagctgggcttcttttggtcctcccccacccaggtgcagtcccgttctccctgcctgggtgagtttgattcctctgccgtggaataggctaggctgctacctcttgagcctcttccaccaggccatccattaggtggcgacagagagcactaaaaggaactactatggaaataaaacttgttttgcttcttggggggaaaaaaaaagaaaaaggcttgtggggcgtgtgtgcattttagtcagattttactgtgcaaaacatttgagagatttctgccctctttctcccttccattcttctcaacccactgggcgccctaccacccctgtctccttcaagataaggtagatcagaagaccaaatagacaaatgccatgtccactgttttctgtcacagttgatagccataccagtcacccaagctggaaacccaacaggcccctgcccttcactgcccacatccaagggagccaccaagtcccacaaattgttcctttaactgtttgtccctcttttgtcttctgtcatcccttctaccgctgtcctggttcaatccctcatcttgctctgggactcccatgataacttatgatctttcctccacctctctatcttccacacaatccctatcatcaatctcattcccctgctttaaacccaagagtggcaccctgtgtttgagtgacatcagggcccctcatgtggctcctgcttctctttgtggccccttctgttgctgctgcttttcttatggacatagccctcagcagtccaggactgcttgtagttcctcccaggtaccatgtttcttgcactcctggcctttgtcattggctcccctgcccaagtccccttctcttctcctttccttcccctgtggccttgccttgtcgtgcttatccttgaagaccctgtcaggtatctcttccccaaagagccctgcctaaccaccgcccccctcccccccgcgacacacacacctgggttaggccctgcctctccacgcctgtgcctcctgccaagtcctcagaggtctctgatcccatgtgcctccaggcatggcatagggggactgtgacacagcctctcggcccacagacccctgattgtgggcttgctcactgccccagtcagtcctcttattgaggattccgtgccagttcctgactccagcacacacacgcatgtaggccgccctcctagtgcctggctccttccctgtctcttctgccactcattcccatggtcgtatcctggagttggtcatctctggaactccacccacggagttctaacttagctctgcctatgatgaggacttactgtcttcccagcttgcagtgtcaaccactgtttgatgcccctgggactccattggtcttccctcctcttgtgaactgtgcccatcaccagacgaacttgttttagaatttaccatcgtaactgagctcccttcagcgcatacctccttggctcctgctcagtctctgtttctccttttagccaaactctctaagagttctctccactcatgggccctcttccttgcctgctgctccttgctcagcttgctccatgaacacttgcttttccacattccatgaaataatcttaacagtcatcagtggctgtcactccttctcagccctttccttgtgtctcttctggtacctcatactctccaggtggccatctcacctcacatcttgaaccctctgggtttgggagaattctcacctcacgagttgatgggaggcctggcgacctctgattgtagtcactgcaaatgccagatgcttatttgcctagcttccctttcggtcagggcagcagttggcaaacggtatctcaagggccaagtccggcccactgcctgttttcgtaaatgaagctttaccaggacccagttccaccccgtcctttgtgcattgtccaagactgctctcctgtacaacagcaggtgggctggttgtgacagatactgtctggcccacaaggtggaaaatactatctggccccttacagaaagaaattacctgagttctacacgagggtgtaggtatgtaccctggcctctgccagtcagactcacatgctaggaggagcagggccaggcaggagagccgtgtctcctggcattggggctgcaggaaagacgagctcctaggccacagtgccagtggccagtgctgctgccttgcagggtcgcacaggcagtgctggctgtttggactggcttggcagaaggatttgaagtattgttcctagccaactggactcaaacctgttcctccaaccctctagggattctcttatcacccagtagccttttccccctagttttaaaaattgcagtaaaatacacaaaagataaaatgtactgccttaaccatttttaagtgtacaattctgtggtattgagcacatttatattgtgcaaccatcaccacatgcatcttcaatagcttttcatcagtccttgtctgcataaatcagctagagttggtttctattgattgccaccaataatcttgacagatatgtctgatcttccttctctgcactgactcctctttctctgtctcctctgctgattctttctcctcatcacaactccaaatagcagggggagggttgtttacacttatattcagcacgccctcacgcactcgcctggctcttcagacctctcccctgaactccagattcatacatccagctgccctttaggcctctagaaagctaaatacctcagtatcaaaaacatgagaaacggaagccagagtcctggatctctcgccctttcgctgtcccggtgcccatgcccttcagggatggcacctagaccagctccctgcatccctgcctagactctgcagtagtctcacgtggcagacccggaggtcactctcctctctggatgccctgcggacactccggttagcctcagctgcaagagcctcctcacccaaggtcacgccatttccaggacagcaccctggtgactgagcgaggtaagggtacaaggcccttatagggccttctctttgacttcttcccacctccctttatggatgtcagttcctgatgaacatcttacacctcaaaccgtgacccaacatctgcttctgcagagcccccctgtggcatcttgtgccctcctgccccactccctctactctatatcttcccatagttagaatgggctttttttttttttttttgagataaggtctccctttgtcacccaggctggaatgcaatggcacagtcacgactcactgcagcctcaacctcctgggctcaagcagtcctcccacctcagcctcccaagtagctgagactacaggtatgcaccaccacacctggctaatttttatattttttgtagagactggggtctccctatgttgcccgggctggtctcgaactcccaggctcaagcaatcctcccgccttggcctcccaaaatgcaggattacaggcgtgtaccagtgtgcccagcctcagatgggctctttgaaaaatgtttattagatcaggttactcccttgagaaaaaccctctcagaataaaacccgaagtccattacttgaaagcagagccagcttcatgggcctttgtaactgcccatgggcttgctggaacccaggcttggtttaatactctactctcaccatctcaaaattcttaatttttgaacaagaggccctgcattttcattttgcaccaggctccacaaattgtgtaactgggcctgcctcagcagccacatggaacatgatccctccttgcctatttgagctcattctctaccattctctcccttgctcacctggctcccactgctcttgctcttcctggaacttgccataatgttgctagagtcagagccttggctcttgctgctcctcattggctggacccctctttacttgacctgctccctcaccactcacttccttcagatctgtgttcagatttcgtcttctcagagaggcttttggcccctgtccatctctctgaatttacctctgacctctcccccaccaccactgcgctaagctgcctcagaactttgtagacattctgtctggtcttctgatgtttcccccttggaagaatcccaaggtgcctgaagaatgctttctttatccttgaagttgagtaggttgactagagtctggcttgctattgagcattctttatcaaattgtcctgggaacatggtgtattctttcagtctgcagatgtagtcgttgctgtttcaggtcagctctcttatggatctttgacagcatcttctgttccatttgttgagttctgtacttcagggacacaaattcctcatgttggattgtctttgtctctcttccaatgctattagctttgccgtaattggtttagcttttgtctttttcatctgcattcactttgtctaatttgattttcagctatgtatattctgtttctggctgtttttcaatgtatttattagtttcataatgatgtgttttggtctgcagtttgtttctctaggttggaaatttgtcttttcatcttattctgttttatcatcccatctttgaactcttttattgggaacatgttcttatgaagttgtggggaatttttttcccttccttgtgtattctcttcttggtgggagactttgcctttctcgtgccatctccctccctgggcctcttttttttcttctggccataatatgtttgcctagttaccatgtcacttcttttcgtcttggctcaggcttggatggctctgcatagtcgttctgtttgctttgagacagtggaggaattcttggctctctcttcccagtttcttggcatcttctcttgctgttttcccctctgagctatcgcgtgcaggcttgttatcttgtatccggagagaatttgcacgctggagggagctgcagccatgtagtcttcagccctatctggattcttctctttgttctaagaactgtgttggatgtcttactaaggctcactctagctgcacgagggatgtgtgtgccatttccatggggatagggggcacctcagtctctgggtggttccataatctgtgtatacctaagagcagttgcttcccacagagctgggctggctcactgggcactttgccatttctcctgcacctcccagctggagtttctgggtctaaaaggaaaaagtgaaggactcccacttggttgcttctctccagcttactgactgcaaattcccagggcgttgcccgctccctagggtggtttctgggggacggggcaggagcctggctttgctgctgctttgtcctctggagtcttttctcagactgctttgaattacacccctttcctttgtgtgctgaaatcttcccttcacactctccttccctgcctttcttttgtgtcttatcttactaggactggaagagggcagttgtgcaggaggtctgcatctaattccctaatccatgtgagagtgctcctgttgtgtgctttgtgacatgatggtgagaaatactccctagagcagtggctaccagaaggaagccatccccccccctgcacacacacacacacacacacacacacacacacacacacacacacactccttctggctgtcctcagatgcctattctaggtaaatgtcagattccaaagaaaatccagttgagatcttttttctttttttgagacgagagtcttgctgtgttgcccaggctggagtgcagtggcacaatctcggctcactgtaacctccgcctcctgggttcaagcgattctcctgcctcagcctcccaagtagctgggactacaggcgcgcaccaccacaccaggctaaaatttttttgtatttttagtagagacagggtttcactgtgttggccaggctggtctcgaactcctgacctcgtgttctgcccgcctcagcctcccagagtgctgggattacaggcttgagccatcgcgcccggcctccagttgggatcttgactggaatgactggtgttcaatcattatagtttccacctaatttgtatttgtacacaggacagttactaatttgttggtacttgtttgatccccagtccctagagttgtttatggggtggagcttcagtccctgctgcttcccctgtggcagcagctggagtcagggtggggacccagggtgctgctggcagattcttgagacaggtagaatctcctctatattggtgtctctctctgtcccagcagtgcccaggaaaacctggccagcctgtcactgacctctccacctagggcactggtggttcaggtccttctatttgccaccggcaaaccgtacttctgccagtctggctcttaggcccagtttctctgatcttgcagattttcttgggctctgctacggaatcctcatacctccggcaggtccctcctttgcccatgtgtttaactgtggtggaatcgtgtgagagctgcttctctcgcatggatcccagccacaccacattctacagcggttcctctgaaggcattgatagagatatttcctcctgttttgcatttcgttggtcatttcagtagaatcagggtgaaataaacatgggggctcagatgtcagcattacgaaccaagtacgtcaggcaggctgatgtggactgacctacactagtgagacgcaagatgacgaaaacaagggcactcactccaagttactgatgagatgtttggatcaaatgagccagtccttaagcagagttctctagtaaaagagatctcctttctgccctttcttgttccccaaaatgtgttgccttcatggtgaaaatttattttggcagattttctcttctttgataaaagcagccaacactttgttaaaagtctgtgaaacttatttacatgaagtatgtaaaggtaagaaaaaaacattatcaacaagaaatggagaaagccagcagctgaggacagaaaagtcatgcacagtgtcagtgtctatggaaacaggccacttggaccttgaggactaggtatttggaattggaggtgagcttggcctggtgagtctctaaccacttgtgtgtaggatcagtgtgagaaccctgctagaatatagtggcagagatgcaaggggaaatcattggagaagttaccagggaatgatgagctaatctgaaaaaaatacatgtttctaagttgggcgtggtagctcatctgtagtcccagctacttgagagcctgaggcaggaggatcgcttgagcccagcctgggcagcacagcgagaccctatctccctaaaaaaaactttttcgttgtttagttttgggatttttttttttcctggtcttttttccccctttttgtgaataacgggatctcactatgttgcccaggcagatctcgaactcctgggcccaagcaatcctcctgcctctgccttcctaagattacaggtatgagccactgtgttaagcaaaaaaacttttttaaatgaaaatcattttttaaaagacaggctttccaggggagggtattattccacttatatgaagtgtcaacagtaggcagatttgtggagacaaatagattagtggttaccaggggctgagaggagtgggagtggggagcaactgcttaatgggtaaagggttgtctttggaactagagagtagtgatggtcgcatgacattgtgaatgtactaaatgctattaatgataaattttatgttatgtgtattttaccacaattaaaaaaaaaagatcaaatgtcctcagaatagccaacaaccttccacttggctaaatgcctactcattaaacttcttgaactaaattcctttctgattgtcatggttattgtgtcctgggcttcagagtttcacattcaggttggcttggtccagtctgtcatgtatcactataggtccccacattggcctcttcctcagacggacagcccatctatctgccggggctctgtgccacagccagatagacttgctctgagacagctgtgtgggctctgagcactggccaggcatcacaaaacctatctttatgatttagaataattggtggtcagctgctgttttaatgttgttgttttttttaatttagatataattcacataccatgaaatttactcatttaaagtgtacaattcattcttcagtataattcataggctcacagaaaaaattgtttaaaaataaaatgtgcaattcagtgtcttttagtacattcacagagttgtgcaaccatcgcctctgtgtcattccagaacactttcagcacccaaaagaaaccccagacacaggagcagtcacctcttattacccgcagcccctggcaacaactcatccacttcctgtctctatggatttgcctattctggacatttcctataaatggaattatgcactatttggccttttgtgtctggcctctttcactgagcgtaatgtcctcaaggttcatctgcattgtagcatgtgtcagaatttctttcctttttgaggctgaatgatattatatcctatagataatgaggttttgattatccacccatcccttgggaatgcatatttgggttgcccccaccatttggctgttgtaaactgtgctgccatgaacactggtgtacggatatctgtttggttactggttttggttttttgtttgtttgttttggttttttgagacaaggtcttgctctgtcgcccaggctggattacagtggcacgatctctgctcactgcaacctccacctcccaggttcaagcaattctcctgcctcagtctcctgagtagctgggactacaggtagcactcaccaccatgcccggctaaatttttttgtatttttagtagagacaaggtttcgccatattggccaggctggtctcaaactcctgacctcaggtgatccacccacctcagcctcccaaagtgctgggattacagacgtgagccaccgcacccggcatagttgtggctttttgagagtgtatggctaggagtaaaattgccaggtcatatggtaactccatgtttaacatttgagaaactgccaaactgttctccacagcaggaattttttaacctgtatgtggtgggcttgtgtttcggttttcattttacacatctataaagatgagatttgctgtatggcactggttgcctgtatttggggagggttctgcttttggttggcaagaactgcattttatttaagcttagcaaaacataactggtttctcgcatcttctcaaaagtggaggattaagaaatggactgcgaattcagagcagggcagctgaacctcaggctccacccttgtagccttcaagctgaacctcattctctcttgctccctggagaccactgagacactctgcctgtgccagtttgatttctcacatttttaaagggccaaagcttgtgtctcaaagtgctatagcctttattgattcatgcagagaagcctccttgattccgtaattctgcagctaatactggaagtagaaagaattggaaacaccatctggatgacactttagggtggaagcagccagtacaagggggggctcattatttcctctggtcccagactgttcacctggagctgtagccaccaccctgcccttaggttaactgcctcgagtggtagtttagctctttgtgctgtgccgagggataactggaagtgaaaggtgctgagaaatgccatctcctgaaagtggcgagcatgagtgaatttacgaaaggttgggatattgctggggctctggaagtttctctggagctcactccaggggacagggagggggctggattccaattcaagtgaaaaatacctttcatctgccttgttcacctggcttttttgcctttttgtaaaatctgaaaacctcagggattgagtagtctttccttaactgcagttgcctgtctggccacacctgccagctgttgcttgtacccctgtaatttgcacggccttccgggcctttctcacaagatcactgcaggtcacattcatgaggaaaatgcaggcagttcctgccatcagacccctcaggatgtcatggtttggcctgaaaacaagattcctgcaactctaattttcctttgctagatcaaatgaaggatttgatctaatgtttgcattctagcagcaaaatcattgaatattttatttcttaagagccttacttcatattttgtaggtattttaagattttgtaaaggcctttctgcttcaacgtgtgatgtgtgcattcttagaaaaagatcttgtgttctgtaaatcacacaataaaaacatgagttcgtgcaggaaaaactggggcggggtggatcactccaaacttgtgtggtgtggtaactggagctcactgatgaaaccatgaacagttctggctgaaagaaccccacagtacactgaggtctgttggcatcgccgccagcaccgccccggtccctttgtgcgcgccaccacacctggctaattttttatttttagtagagagggggtttcaccatgttggtcaggatggcctcgaactgacctcgtgatccgcccacctcagcctcccaaagtgctgggattacaggtgtgagcctccgtgcccagccttcagctttttttcttaatgtctttgtgtaatatgaaggcattctctttaattgttaaaaagcttgcctaccactgcttcaaaatattactgtcagttggcatagcttctgattatattgatgtcatctcccttcttttaaacatgttaccatattggcactgtatttcccctagcccattgatcacttgagagttagtcatagtcctcgtgctgtttcactcctaaacgtttaagcatgcctttcctaagagcagacagtacagttaagacactcaggaagtttagcaatgagctaacacagaaccttacatttctccacataccccataaatgccttttttagagcctttgagcctggaatgcagagtccaggactgtgtgttgtattcgattgtgtcatcccttcagtctcctttatcagaaatgttcccccacccccttgttttctctcatcatcttgagtccagaccgtggttgcatggcacgccctctctggactcttcctgctgtctcctcacggtaagcttcagtctcctactcgtgatgctggttcatctcagcagcactgaggggcctgagctcagtttggtcgtgtgttaaggtggtgcctgccagatttctccacagaaaagggccccgtacttttatttgctcttcagcctgtgtattccttcctttcttgccagcttgtgggtggcttctctagcagcttctgtaagatactcagtttggcagttgtagttgtttcagcaggagaggtgtctgcatacctgaccaccacatggctagaagtcgatccatcctctggcgtaaccatcctccatgctactgtccctggggcactgaggccctcctcagtgacttcctccacctcatcttccgccatctccaagccaccagtgtccaacggactactgatatgtcccaaactcatcatttgtttattcaccaattcagagcccacctttttttcagcactgagctagcctctccttgctagaagcttacggtcgaaggtctccagccatcagaagaagcacgtggagcgctgcgtccgtgttgtggttattcatccagcatgtgttgagtaagggttgcacctgtgcctggcattatgcattgagcggggagatgggggttggcacgcacagtggggtgttctaagtacactgagggctcgggtgccctggctcatagagcagggagggaggcaggagcagggaaggtgtctcagaagtgccatctttttttttttttttttgggaagtggaatcttgttctatcgcctggtctggagtgcaatggcactatctcaactcactgcagcctccgcctcccaggttcaagcgattctcatgcctcagtccccgagtagctgggaccacaggcgcacaccaccacacccggcaaatattttgtatttttagtagaggcggagttttgccatgttggccaggctggtcttaaactcctggcctcaagtgatctgctcacctcggcctcctaaggtgttgggattacaggcatgagccactgcgcccggtctagaagtgccatcctaactgaacctgaaagatgaaagttctccagatgaacctgaaagttctccaaatgaaaaggtgggagggggtgacagggttaggcccagagcctctggtgacacagggtgggcatcattggtcactttttcctcgagggaggggcgtcacacgggtgatagggtgggagctataaccatgttgatagtgccgcctctgcccatctggcctggcatgccctgagccctctgtcccacctgtggaactcataagccctgacagcccactcactcctgattcattatccacacccctgtgcttccgctgtgcctggagcaagctttcttcagggggaagggaggctggaactatgttgtagttacctatttgtcctcccttccaaactgtgagttcttggaggtggaaggatgctgcaggatctggctcaggacgaaggcagttggtgaacagacacgtgtgtttttgactcacggtgatctcagacaagttcctctgtctagtcgaacttctttttttccatctgtaacactcaggagttgaataggtggtttttctgaggatacttcaactgtaaaatgtatgaacttgtgaactagctatttagttctcctcataatcaagattgtgtgtgtgtggggggttctgattagagggaggatgaagagaggtgtatggggttttttttgttttgttttctgtttgtttgtttgtttttgagatggagtctcactctgtcacccaggctggagtgcagtggcacgatttcggttcactgcaacctctgcctcctgggttcaagtgattctcctgcctcagcctcctgagtaactgggattacaggcatgcaccaccatgcccagctaatttttgtatttttaatagagatggggttttcgccatgttggccaggctggtctcgaactcctgacctcaggtgatccacctgcctcggcctcccaaagtgctgggattataggcatgagccaccacacctggcaggtttctttgaaaaagtttgtgtttcggcaaacaccataaaccccctgggggacagccttggggagtcacctggcaccctagcccagcctccctcccttgggtcctgcagtgaaggcttagtgagggtgtgcaaatgcccaggtcaccctgggactgggcaggccctctgggctaagggtaaactcatttggaatacctgttttctatcattgttttttatttgttaaatttaaagggtacaagtgcagttttgttgcgtggatatattgtatagtagtgaagtctgagctttcagtgtaaccatcacctgaatagtggacattgtacccgttaagtaatgtctcatccctcaccccctcccacccttcccagtctctccagtgtctgccattcctcactctgtccatgtgcacatgctattcagctcctgcttctaagtgagaacgtacggtatttgactttctgtgtctgagctgtgtcactgaagacaatggactccagctccatccacgttttttatcatttttacctgcactccacacccagcacaatccaggcttctttgtgggttttttgaaatttgtctttaattataaaagtagcagccagcaaattaacaaacacccatgtgcctttcattgcacagaattgaaaatcatcatactatatttgcttcaagtaatttccattagaaagaactagaatattacagtagagttaaagaccctttatttcccatcttcagtgctcttaaaagttcatttagggccaggcatggtggctcacacctataatcccagcactttgagaggcccaggtgggtggatcacctgaggtcaggagttcaagaccagcctggccaacatggcgaaaccccatctctactaaaaatacaaaaattagctgggcgtggtggtgcgcatctgtaatctcagctactcgggaggctgaggcaggagaatcgcttgaactcaggagggaggcagagcctgtatgcagtaagccgagattgcgccaccacaccccagcatgggtgacagagcaagactccgtctcaaaaaaaaaaaaaaaaaagttcattcattgtacacttagaaatagttaaaaaggtaaactttgttttgtgtgtgtgtgtatatatatatatatatatatatatatatatatatatatatatgtatttttttttgagacatatatgtgtctggtttgttcgcccaggcaggagtgcagtggcatgatcaacggctcactgcagcctcaacttcctaggctcaagtgatcctcctgcctcagcctcccgagtagctaggattacaggcacacaccaccatgcccagctaattttttttttttttttttttttttgtagagacagggttttgctatgttgcccaggctggtctcaaactcctgagctcaagcgatccacctgcctcacctcccaaagtgctgggattacaagtgtaagccaccacacctgacctgttttgtatattttaccacaataaaaagcctttaaaaccccaagcagacagttcattttcattcaggcccaactcagaatctgatcacagcggggtttcccccctttctagcgagtagctgaagaactgttttctctccttgatggtataactgtctctgtgggtgttgctcccctgccgctccagtggttttgtttttgtttttgtttttttgagacggagtcttgcgatctcagctcactgcgacctctgcctcctgggttcaggcgattcttctccctcagccttccatgtagctgggacttacaggcacctgccaccacgcccggctcatttttgtatttttagtagagacggagtttcaccatgttggccaggttgggctcgaactccagacctcaggtgatccacctgcctcagcctcccacagtgctgggattacaggtgagagccactgcacccagccggcccctcagtcttttccttctcaatcagtggcaccaccatcttcccaggctttggacatggtccctgactcacccttgcccctcacccccacactaatccacctgcgagctctgttgcttcaccacctagaccagccccaaatcctcaactgcccccaccctgggccacacctggaccactgctagaggcctctcatgggccctccctgtttttctcttgcactccccgggctttctggcacaagatgccccagaagcagaatcacatatctctcctgggagccaatctagtgtgtttactgcccctggagtgttattgttggccttagaatatgtcccactacaggtttgcagagcactgtagtcaaaagtcatttgaaataaatcttttctctgtggtatattgtcaatttgatatagaattaaatttgtttcttttcttttttcttttctttttttttttttttaagagacagggtcttggccaggcgtggtgtctcatgcctgtaatcccggcactttgggaagccaaggtgggtggatcgcctgaggtcaggaattcaagaccaacctggccagcatggtgaaaccccgtctctgctaaaaatacaaaaattagccgggcgtgatggcaggtacctgtaatcccagctactcgggaagctgaggcaggagaaggcttgaactcaggagtcggaggttgcagtgagccaagatcacgccatggcactctagcaagactctgtctcaaaaaaaaaaaaagagagagagagagacagggtcttgctctgtcactcaggctggagtgcagtgatgtagtcatggctcactgcagcctcatactcctgacctcaggtgatcgacccgcctcggcctcccaaagtgctgggatcgtaggctgaagccaccatgcctggcccgaactcatttgtttttatttgcattaagtgtaataaggttttgttacttttagtttgaattttattttgggtaatataaacatttacatgattcagaagtcagaattacactgaggcatgttcagctaggcctcactcctgtgcctgtacccttacctttttccccctaccccatgcagggaatcaatttcattagttcctggtgtgtccttccttaatacccccccttctttctttggtagaatgcagtagatatgtttgcgctttgctccctttgcttcacagtggatcctggaaatgactccatcgcagttcttagagctcttgtttagtccctttggatctgcacagtactccagtgtgtgggcgcaccataagtttattcagcaagtgccctggtgatagggatcgggggtattggaagcctttggctggtaaaaataatgttgtagcaaataacatcatgcatatgttctttgagatttctggaggtgtctctttagcatagatttctagaaggcattccttacgtcacgtttaggtttatagtttgacctcatggtgattaaggtatttgggaaatgcaaatgagagtttcgaagaagccagatctttcccattagttcactgtttttctctgacattaggaccgtccgggttctagggagcagccctggcgttaggcagtgccatgatggattgtgtagaagtagcgattcccatctgtctgctttcttggcccactctgctggtggctccccttccctccctcctttatggggagctggggagctgcctaggggtccattctcaaaggctgatctctggtgggcaacaggccacacctagctttccagggttcttcgtcatttcccattgagagctgtaagactcagagacatgaaaaggaagctctggctgggcacggtggctcacgcctgtaatcccagcactttgggaggctgaggcgggtcgatcacctgaggtcaggagttcgagaccagcctgcccaacatggtgaaaccccgtctccactaaacatacaaaaattagcctggcgtggtagcacacgcctgtgatcccagctactccggaggctgaggcaggagaataacttgaacccggcaggcggaggttgcgatgagccgatattatgccatcggcaacagagcgagactccatctcaaaaaaaaaacaaaaaacaaaacaaggcgagctctgtgctgggacagattagggacccctctttacagcaagaaagactgctctgtgggttgtaggatgcctttgtgtatgcagtggctctaggtgactctggcagccacactctgggccctaaacttctggaggaagatacaggatagggaggaactcaggggtgagtcatggtggggacaagacattccctcactctaagaccttgtcactagattggaacatctcttgcctccctacacctgacctgatggttctggagagatacgtccttgcagcttctgagtcccagcactaagcagcctttggtaacttccctacatcatttgagttctggtttcctaaggatgcttgccagtgagtgccatggtgccctcattgcacagtctgtgcagtgtagacaagaggggaagtctcttggggtagaccagccgcaaggcggtgactagcactgatgtgaaccacatgggacaggggagttgtggggctgagaacacggagggtgggagtagtcatgctcttttccagaatgaactgctaacgaagggactcgcaggtggctgctgcttctttccaagctgcccctgttgttgcagaggctctggagtcctaggaggtttcacggtggcatactcgacagagtactagagcatcatggccagatagtgatgctggggtgtggggcctcacggtggccatttctgacgagaccccaccgggccaaagtgatgtgtagagaaggagctgcttcggtcaccagaaaagaacggggaagcctcccacactagaataggtagggtgctcttctccaccggcaggaaggggatgtatggctctgcctggaccacacctttttccttgctcttccctccgcatctgctgtggccgaggccattcctcatcagggaacatgtgttagaggctcacgccacctgggaccacttgtcttatcacccccaggaccctaggcggtagtttcctgtggcctgagttagctgatatttatatagtgccattgtgccttttctcctgtgatgctcacagtaaggatgcctagatggggttacctgttgtcaagataaggaaactgaagcacagaatgctgaggtcatttgctgggttcatgtttggaaagcggcaaaggatttcagtgcaggttggctggctccaaacctgtgtgtgctttccatgacactgtactgtgtgcctcattgagcctcattctagaaaaccaaaaacacacccaaggcccggccttcacaaaggagacccctcccccatttggctccctttccagcagtcgacggcctcttgtcagccatcgagcccagagtcccttgaagtgcgactcatgctggggtggtatgctcaggagccgcagtgtttccgctcagaggaaagggctctgattctcctgcagtgctaggagacttgtgggtggccacagtgcaggtcaggcacaccggccagcaccacccacagcccaaattcctaaagaaatatttgggtcccagcttggcccgagtctctgttgtcctggggaaggacatcaagatctgagtgtatgatggcctggggccttgcatgtggtgggggtccaagcctgcctctgctcacttgttctgcagactggcatgttctctgtgatacttacatacttgtttaacacttcagggaagaaaagtcagaagaccaggacctccagggcctcaaggacaaacccctcaagtttaaaaaggtgaagaaagataagaaagaagagaaagagggcaagcatgagcccgtgcagccatcagcccaccactctgctgagcccgcagaggcaggcaaagcagagacatcagaagggtcaggctccgccccggctgtgccggaagcttctgcctcccccaaacagcggcgctccatcatccgtgaccggggacccatgtatgatgaccccaccctgcctgaaggctggacacggaagcttaagcaaaggaaatctggccgctctgctgggaagtatgatgtgtatttgatcaagtaagtaagagcaactcctatctctacagggcagggagggcagggacaaggatccctcatggagcaggaaaatgtatgtgcccagggtggggtcggggggaacataaacaatgaacactgagaccaggtgtgcttgaaatgaccgtgtacagaggtcgctgccctgagtgggaagttctcaaggtagcaggccctctatcctctccacacctcaagtctttatctggggatggaatagctgcggaagcagaggaacttgcagagctaggggttcagaggggtgaagaagcatgtttcagttctgccttttaaatgatcccaaaaaggttagcagttttcaaatgacatttgcagacagcctcatttaattccatgagaagggtgagcaaaggattatcttgttgaaactgattcctggagagactgagcaccgtacctgagttcaaacttgggaatgttctagatggtgactcaggcccaggcaccaaccagcagaatgggcctcagcctgacaacccttctgtaccaggcctgactctttggttgctgaactttggagaggcctgggggggtcagcggcaggcagacgagtgagtggctttggtgacaggtcctcaggggcagccaggcagtgtgactctcgttcaatagtaacgtttgtcagagcgttgtcaccaccatccgctctgccctatctctgacattgctatggagagcctctaattgttccttgtgtctttctgtttgtccccacagtccccagggaaaagcctttcgctctaaagtggagttgattgcgtacttcgaaaaggtaggcgacacatccctggaccctaatgattttgacttcacggtaactgggagagggagcccctcccggcgagagcagaaaccacctaagaagcccaaatctcccaaagctccaggaactggcagaggccggggacgccccaaagggagcggcaccacgagacccaaggcggccacgtcagagggtgtgcaggtgaaaagggtcctggagaaaagtcctgggaagctccttgtcaagatgccttttcaaacttcgccagggggcaaggctgaggggggtggggccaccacatccacccaggtcatggtgatcaaacgccccggcaggaagcgaaaagctgaggccgaccctcaggccattcccaagaaacggggccgaaagccggggagtgtggtggcagccgctgccgccgaggccaaaaagaaagccgtgaaggagtcttctatccgatctgtgcaggagaccgtactccccatcaagaagcgcaagacccgggagacggtcagcatcgaggtcaaggaagtggtgaagcccctgctggtgtccaccctcggtgagaagagcgggaaaggactgaagacctgtaagagccctgggcggaaaagcaaggagagcagccccaaggggcgcagcagcagcgcctcctcaccccccaagaaggagcaccaccaccatcaccaccactcagagtccccaaaggcccccgtgccactgctcccacccctgcccccacctccacctgagcccgagagctccgaggaccccaccagcccccctgagccccaggacttgagcagcagcgtctgcaaagaggagaagatgcccagaggaggctcactggagagcgacggctgccccaaggagccagctaagactcagcccgcggttgccaccgccgccacggccgcagaaaagtacaaacaccgaggggagggagagcgcaaagacattgtttcatcctccatgccaaggccaaacagagaggagcctgtggacagccggacgcccgtgaccgagagagttagctgactttacacggagcggattgcaaagcaaaccaacaagaataaaggcagctgttgtctcttctccttatgggtagggctctgacaaagcttcccgattaactgaaataaaaaatatttttttttctttcagtaaacttagagtttcgtggcttcagggtgggagtagttggagcattggggatgtttttcttaccgacaagcacagtcaggttgaagacctaaccagggccagaagtagctttgcacttttctaaactaggctccttcaacaaggcttgctgcagatactactgaccagacaagctgttgaccaggcacctcccctcccgcccaaacctttcccccatgtggtcgttagagacagagcgacagagcagttgagaggacactcccgttttcggtgccatcagtgccccgtctacagctcccccagctccccccacctcccccactcccaaccacgttgggacagggaggtgtgaggcaggagagacagttggattctttagagaagatggatatgaccagtggctatggcctgtgcgatcccacccgtggtggctcaagtctggccccacaccagccccaatccaaaactggcaaggacgcttcacaggacaggaaagtggcacctgtctgctccagctctggcatggctaggaggggggagtcccttgaactactgggtgtagactggcctgaaccacaggagaggatggcccagggtgaggtggcatggtccattctcaagggacgtcctccaacgggtggcgctagaggccatggaggcagtaggacaaggtgcaggcaggctggcctggggtcaggccgggcagagcacagcggggtgagagggattcctaatcactcagagcagtctgtgacttagtggacaggggagggggcaaagggggaggagaagaaaatgttcttccagttactttccaattctcctttagggacagcttagaattatttgcactattgagtcttcatgttcccacttcaaaacaaacagatgctctgagagcaaactggcttgaattggtgacatttagtccctcaagccaccagatgtgacagtgttgagaactacctggatttgtatatatacctgcgcttgttttaaagtgggctcagcacatagggttcccacgaagctccgaaactctaagtgtttgctgcaattttataaggacttcctgattggtttctcttctccccttccatttctgccttttgttcatttcatcctttcacttctttcccttcctccatcctcctccttcctagttcatcccttctcttccaggcagccgcggtgcccaaccacacttgtcggctccagtccccagaactctgcctgccctttgtcctcctgctgccagtaccagccccaccctgttttgagccctgaggaggccttgggctctgctgagtccgacctggcctgtctgtgaagagcaagagagcagcaaggtcttgctctcctaggtagccccctcttccctggtaagaaaaagcaaaaggcatttcccaccctgaacaacgagccttttcacccttctactctagagaagtggactggaggagctgggcccgatttggtagttgaggaaagcacagaggcctcctgtggcctgccagtcatcgagtggcccaacaggggctccatgccagccgaccttgacctcactcagaagtccagagtctagcgtagtgcagcagggcagtagcggtaccaatgcagaactcccaagacccgagctgggaccagtacctgggtccccagcccttcctctgctcccccttttccctcggagttcttcttgaatggcaatgttttgcttttgctcgatgcagacagggggccagaacaccacacatttcactgtctgtctggtccatagctgtggtgtaggggcttagaggcatgggcttgctgtgggtttttaattgatcagttttcatgtgggatcccatctttttaacctctgttcaggaagtccttatctagctgcatatcttcatcatattggtatatccttttctgtgtttacagagatgtctcttatatctaaatctgtccaactgagaagtaccttatcaaagtagcaaatgagacagcagtcttatgcttccagaaacacccacaggcatgtcccatgtgagctgctgccatgaactgtcaagtgtgtgttgtcttgtgtatttcagttattgtccctggcttccttactatggtgtaatcatgaaggagtgaaacatcatagaaactgtctagcacttccttgccagtctttagtgatcaggaaccatagttgacagttccaatcagtagcttaagaaaaaaccgtgtttgtctcttctggaatggttagaagtgagggagtttgccccgttctgtttgtagagtctcatagttggactttctagcatatatgtgtccatttccttatgctgtaaaagcaagtcctgcaaccaaactcccatcagcccaatccctgatccctgatcccttccacctgctctgctgatgacccccccagcttcacttctgactcttccccaggaagggaaggggggtcagaagagagggtgagtcctccagaactcttcctccaaggacagaaggctcctgcccccatagtggcctcgaactcctggcactaccaaaggacacttatccacgagagcgcagcatccgaccaggttgtcactgagaagatgtttattttggtcagttgggtttttatgtattatacttagtcaaatgtaatgtggcttctggaatcattgtccagagctgcttccccgtcacctgggcgtcatctggtcctggtaagaggagtgcgtggcccaccaggcccccctgtcacccatgacagttcattcagggccgatggggcagtcgtggttgggaacacagcatttcaagcgtcactttatttcattcgggccccacctgcagctccctcaaagaggcagttgcccagcctctttcccttccagtttattccagagctgccagtggggcctgaggctccttagggttttctctctatttccccctttcttcctcattccctcgtctttcccaaaggcatcacgagtcagtcgcctttcagcaggcagccttggcggtttatcgccctggcaggcaggggccctgcagctctcatgctgcccctgccttggggtcaggttgacaggaggttggagggaaagccttaagctgcaggattctcaccagctgtgtccggcccagttttggggtgtgacctcaatttcaattttgtctgtacttgaacattatgaagatgggggcctctttcagtgaatttgtgaacagcagaattgaccgacagctttccagtacccatggggctaggtcattaaggccacatccacagtctcccccacccttgttccagttgttagttactacctcctctcctgacaatactgtatgtcgtcgagctccccccaggtctacccctcccggccctgcctgctggtgggcttgtcatagccagtgggattgccggtcttgacagctcagtgagctggagatacttggtcacagccaggcgctagcacagctcccttctgttgatgctgtattcccatatcaaaagacacaggggacacccagaaacgccacatcccccaatccatcagtgccaaactagccaacggccccagcttctcagctcgctggatggcggaagctgctactcgtgagcgccagtgcgggtgcagacaatcttctgttgggtggcatcattccaggcccgaagcatgaacagtgcacctgggacagggagcagccccaaattgtcacctgcttctctgcccagcttttcattgctgtgacagtgatggcgaaagagggtaataaccagacacaaactgccaagttgggtggagaaaggagtttctttagctgacagaatctctgaattttaaatcacttagtaagcggctcaagcccaggagggagcagagggatacgagcggagtcccctgcgcgggaccatctggaattggtttagcccaagtggagcctgacagccagaactctgtgtcccccgtctaaccacagctccttttccagagcattccagtcaggctctctgggctgactgggccaggggaggttacaggtaccagttctttaagaagatctttgggcatatacatttttagcctgtgtcattgccccaaatggattcctgtttcaagttcacacctgcagattctaggacctgtgtcctagacttcagggagtcagctgtttctagagttcctaccatggagtgggtctggaggacctgcccggtgggggggcagagccctgctccctccgggtcttcctactcttctctctgctctgacgggatttgttgattctctccattttggtgtctttctcttttagatattgtatcaatctttagaaaaggcatagtctacttgttataaatcgttaggatactgcctcccccagggtctaaaattacatattagaggggaaaagctgaacactgaagtcagttctcaacaatttagaaggaaaacctagaaaacatttggcagaaaattacatttcgatgtttttgaatgaatacgagcaagcttttacaacagtgctgatctaaaaatacttagcacttggcctgagatgcctggtgagcattacaggcaaggggaatctggaggtagccgacctgaggacatggcttctgaacctgtcttttgggagtggtatggaaggtggagcgttcaccagtgacctggaaggcccagcaccaccctccttcccactcttctcatcttgacagagcctgccccagcgctgacgtgtcaggaaaacacccagggaactaggaaggcacttctgcctgaggggcagcctgccttgcccactcctgctctgctcgcctcggatcagctgagccttctgagctggcctctcactgcctccccaaggccccctgcctgccctgtcaggaggcagaaggaagcaggtgtgagggcagtgcaaggagggagcacaacccccagctcccgctccgggctccgacttgtgcacaggcagagcccagaccctggaggaaatcctacctttgaattcaagaacatttggggaatttggaaatctctttgcccccaaacccccattctgtcctacctttaatcaggtcctgctcagcagtgagagcagatgaggtgaaaaggccaagaggtttggctcctgcccactgatagcccctctccccgcagtgtttgtgtgtcaagtggcaaagctgttcttcctggtgaccctgattatatccagtaacacatagactgtgcgcataggcctgctttgtctcctctatcctgggcttttgttttgctttttagttttgcttttagtttttctgtcccttttatttaacgcaccgactagacacacaaagcagttgaatttttatatatatatctgtatattgcacaattataaactcattttgcttgtggctccacacacacaaaaaaagacctgttaaaattatacctgttgcttaattacaatatttctgataaccatagcataggacaagggaaaataaaaaaagaaaaaaaagaaaaaaaaacgacaaatctgtctgctggtcacttcttctgtccaagcagattcgtggtcttttcctcgcttctttcaagggctttcctgtgccaggtgaaggaggctccaggcagcacccaggttttgcactcttgtttctcccgtgcttgtgaaagaggtcccaaggttctgggtgcaggagcgctcccttgacctgctgaagtccggaacgtagtcggcacagcctggtcgccttccacctctgggagctggagtccactggggtggcctgactcccccagtccccttcccgtgacctggtcagggtgagcccatgtggagtcagcctcgcaggcctccctgccagtagggtccgagtgtgtttcatccttcccactctgtcgagcctgggggctggagcggagacgggaggcctggcctgtctcggaacctgtgagctgcaccaggtagaacgccagggaccccagaatcatgtgcgtcagtccaaggggtcccctccaggagtagtgaagactccagaaatgtccctttcttctcccccatcctacgagtaattgcatttgcttttgtaattcttaatgagcaatatctgctagagagtttagctgtaacagttctttttgatcatctttttttaataattagaaacaccaaaaaaatccagaaacttgttcttccaaagcagagagcattataatcaccagggccaaaagcttccctccctgctgtcattgcttcttctgaggcctgaatccaaaagaaaaacagccataggccctttcagtggccgggctacccgtgagcccttcggaggaccagggctggggcagcctctgggcccacatccggggccagctccggcgtgtgttcagtgttagcagtgggtcatgatgctctttcccacccagcctgggataggggcagaggaggcgaggaggccgttgccgctgatgtttggccgtgaacaggtgggtgtctgcgtgcgtccacgtgcgtgttttctgactgacatgaaatcgacgcccgagttagcctcacccggtgacctctagccctgcccggatggagcggggcccacccggttcagtgtttctggggagctggacagtggagtgcaaaaggcttgcagaacttgaagcctgctccttcccttgctaccacggcctcctttccgtttgatttgtcactgcttcaatcaataacagccgctccagagtcagtagtcaatgaatatatgaccaaatatcaccaggactgttactcaatgtgtgccgagcccttgcccatgctgggctcccgtgtatctggacactgtaacgtgtgctgtgtttgctccccttccccttccttctttgccctttacttgtctttctggggtttttctgtttgggtttggtttggtttttatttctccttttgtgttccaaacatgaggttctctctactggtcctcttaactgtggtgttgaggcttatatttgtgtaatttttggtgggtgaaaggaattttgctaagtaaatctcttctgtgtttgaactgaagtctgtattgtaactatgtttaaagtaattgttccagagacaaatatttctagacactttttctttacaaacaaaagcattcggagggagggggatggtgactgagatgagaggggagagctgaacagatgacccctgcccagatcagccagaagccacccaaagcagtggagcccaggagtcccactccaagccagcaagccgaatagctgatgtgttgccactttccaagtcactgcaaaaccaggttttgttccgcccagtggattcttgttttgcttcccctccccccgagattattaccaccatcccgtgcttttaaggaaaggcaagattgatgtttccttgaggggagccaggaggggatgtgtgtgtgcagagctgaagagctggggagaatggggctgggcccacccaagcaggaggctgggacgctctgctgtgggcacaggtcaggctaatgttggcagatgcagctcttcctggacaggccaggtggtgggcattctctctccaaggtgtgccccgtgggcattactgtttaagacacttccgtcacatcccaccccatcctccagggctcaacactgtgacatctctattccccaccctccccttcccagggcaataaaatgaccatggagggggcttgcactctcttggctgtcacccgatcgccagcaaaacttagatgtgagaaaaccccttcccattccatggcgaaaacatctccttagaaaagccattaccctcattaggcatggttttgggctcccaaaacacctgacagcccctccctcctctgagaggcggagagtgctgactgtagtgaccattgcatgccgggtgcagcatctggaagagctaggcagggtgtctgccccctcctgagttgaagtcatgctcccctgtgccagcccagaggccgagagctatggacagcattgccagtaacacaggccaccctgtgcagaagggagctggctccagcctggaaacctgtctgaggttgggagaggtgcacttggggcacagggagaggccgggacacacttagctggagatgtctctaaaagccctgtatcgtattcaccttcagtttttgtgttttgggacaattactttagaaaataagtaggtcgttttaaaaacaaaaattattgattgcttttttgtagtgttcagaaaaaaggttctttgtgtatagccaaatgactgaaagcactgatatatttaaaaacaaaaggcaatttattaaggaaatttgtaccatttcagtaaacctgtctgaatgtacctgtatacgtttcaaaaacaccccccccccactgaatccctgtaacctatttattatataaagagtttgccttataaatttacataaaaatgtccgtttgtgtcttttgttgtaaaaatcaagtgattttttcataaggttcttttactattggaaaagatgggcagcacgcagttttattttatttttgtaagttttttaatacatgtgaaagcaaagaatactcagcatgcctttctaagtgacgcgtttgcaccttttgttgggaagtactgtatcctgtgctgttagcattctcgataaatctctctgtgaaagtgactcaaggtctgggctttcattataagacagaagtccccctccagctcacatgacagcatggtgctgcgtttcctcattggatctggctgtccctggacacaggtagctgccttcaggcctgccacgagcggccaagggaagcctcctccatatgctggcctcgctggcccctcagcttcttccaagccagtgctctccaggcacactgctccagcgtgtgacgggaagggcctggcatgagtcagcctgcagcacaacctccctgctccagacccgtatggtaggggcaccccctaggtctggatgtgctgtggtgcttttggacacccccacccccgcaggctgtggctcctcctgtgtctcattctggccaggaccctcacgtgccctctgttgactgctaacgtggttctctgaccaggcaagggcaggctgaggggtttgcccaaagggggcccccttgttactggcttccttggctctcaggagcagcctcaccaggttggtaaggggctggaggagacaactgctcaaaggagtccagcttcacatgcacatgctagaaggtaccctcggaaggcctggccttcaaaggtagatcccagggttgaaaagtcaacttgtatgcattgagcatctcgtatgccagccctgttccgtgagctgatgggcctttgtgtgtaagtaggaccaagtgcccccgtggaggttagcatgggtgtgcagtcatttcagatacttgagttggtacatctcagtaaagtctgtcccgtgagaagccatgggtttcatggtatggttggcatcttccttgggagtggccacagtggtggtggcttcaggaaagagactccaacaggggccagctgtgggccttgggcacttctcgtttctaggaaaagtcctaagtctgtagggctaggggtggggaaccccttcgctgtcaggatcaagagggcaaggggaactgtcgctggaggagacatccagctggagaaacaaaagagtaagtctgcgttgctgcttgtggggtcttccccatctcagggcggggaccgggggtggcggtccagacaagtaatcaaggacgatgcccaggaggggacaggtacggggtggcaggagctctgccggcgggctcaggaagccttcaccacagctgcctgagctcacccttgccaaatgagggctggggcagcagcaacgcatacactcacggctgtggcgggcagcgttctcggcatatttcaggacacctaaggagactgaatggctcaaggctgctgccgtgtgcagggggctagacgtggggcgggcaggcagggctcctggtaacagccctgcaggccgcagtggagagcagggttccggcagggccgcccaggagctttcggaaggcccggccccggcccctttccgagcagcccgggcctccgccctgccctctgtccccaacgccgggagccgccgttcgtcctccagagccccgcccgggcgagcccgggaggccgatcgccgctcgcggaacccgccgggacccgggccctccccggcgcggggcgcccccgtgtgacccagcgcgcggccgcggcgcgcaagatggcggcgggcccgggcaccgccccttccgccccgccgggcgtcgcacgaggccggctcgaaggggaagtgagtcagtgtccgcggacccggccggcccaggcccgcgcccgccgcggccctgagaggccccggcaggtcccggcccggcggcggcagccatggccggggggccgggcccgggggagcccgcagcccccggcgcccagcacttcttgtacgaggtgccgccctgggtcatgtgccgcttctacaaagtgatggacgccctggagcccgccgactggtgccagttcggtgggtggcggcgggctgccggggggcgggaggcgcgcgggctcctggcgccgacgcctgacgccc

SEQ ID NO: 2 - DNA, 10241 bp, Homo sapiens
ccggcgtcggcggcgcgcgcgctccctcctctcggagagagggctgtggtaaaagccgtccggaaaatggccgccgccgccgccgccgcgccgagcggaggaggaggaggaggcgaggaggagagactgctccataaaaatacagactcaccagttcctgctttgatgtgacatgtgactccccagaatacaccttgcttctgtagaccagctccaacaggattccatggtagctgggatgttagggctcagggaagaaaagtcagaagaccaggacctccagggcctcaaggacaaacccctcaagtttaaaaaggtgaagaaagataagaaagaagagaaagagggcaagcatgagcccgtgcagccatcagcccaccactctgctgagcccgcagaggcaggcaaagcagagacatcagaagggtcaggctccgccccggctgtgccggaagcttctgcctcccccaaacagcggcgctccatcatccgtgaccggggacccatgtatgatgaccccaccctgcctgaaggctggacacggaagcttaagcaaaggaaatctggccgctctgctgggaagtatgatgtgtatttgatcaatccccagggaaaagcctttcgctctaaagtggagttgattgcgtacttcgaaaaggtaggcgacacatccctggaccctaatgattttgacttcacggtaactgggagagggagcccctcccggcgagagcagaaaccacctaagaagcccaaatctcccaaagctccaggaactggcagaggccggggacgccccaaagggagcggcaccacgagacccaaggcggccacgtcagagggtgtgcaggtgaaaagggtcctggagaaaagtcctgggaagctccttgtcaagatgccttttcaaacttcgccagggggcaaggctgaggggggtggggccaccacatccacccaggtcatggtgatcaaacgccccggcaggaagcgaaaagctgaggccgaccctcaggccattcccaagaaacggggccgaaagccggggagtgtggtggcagccgctgccgccgaggccaaaaagaaagccgtgaaggagtcttctatccgatctgtgcaggagaccgtactccccatcaagaagcgcaagacccgggagacggtcagcatcgaggtcaaggaagtggtgaagcccctgctggtgtccaccctcggtgagaagagcgggaaaggactgaagacctgtaagagccctgggcggaaaagcaaggagagcagccccaaggggcgcagcagcagcgcctcctcaccccccaagaaggagcaccaccaccatcaccaccactcagagtccccaaaggcccccgtgccactgctcccacccctgcccccacctccacctgagcccgagagctccgaggaccccaccagcccccctgagccccaggacttgagcagcagcgtctgcaaagaggagaagatgcccagaggaggctcactggagagcgacggctgccccaaggagccagctaagactcagcccgcggttgccaccgccgccacggccgcagaaaagtacaaacaccgaggggagggagagcgcaaagacattgtttcatcctccatgccaaggccaaacagagaggagcctgtggacagccggacgcccgtgaccgagagagttagctgactttacacggagcggattgcaaagcaaaccaacaagaataaaggcagctgttgtctcttctccttatgggtagggctctgacaaagcttcccgattaactgaaataaaaaatatttttttttctttcagtaaacttagagtttcgtggcttcagggtgggagtagttggagcattggggatgtttttcttaccgacaagcacagtcaggttgaagacctaaccagggccagaagtagctttgcacttttctaaactaggctccttcaacaaggcttgctgcagatactactgaccagacaagctgttgaccaggcacctcccctcccgcccaaacctttcccccatgtggtcgttagagacagagcgacagagcagttgagaggacactcccgttttcggtgccatcagtgccccgtctacagctcccccagctccccccacctcccccactcccaaccacgttgggacagggaggtgtgaggcaggagagacagttggattctttagagaagatggatatgaccagtggctatggcctgtgcgatcccacccgtggtggctcaagtctggccccacaccagccccaatccaaaactggcaaggacgcttcacaggacaggaaagtggcacctgtctgctccagctctggcatggctaggaggggggagtcccttgaactactgggtgtagactggcctgaaccacaggagaggatggcccagggtgaggtggcatggtccattctcaagggacgtcctccaacgggtggcgctagaggccatggaggcagtaggacaaggtgcaggcaggctggcctggggtcaggccgggcagagcacagcggggtgagagggattcctaatcactcagagcagtctgtgacttagtggacaggggagggggcaaagggggaggagaagaaaatgttcttccagttactttccaattctcctttagggacagcttagaattatttgcactattgagtcttcatgttcccacttcaaaacaaacagatgctctgagagcaaactggcttgaattggtgacatttagtccctcaagccaccagatgtgacagtgttgagaactacctggatttgtatatatacctgcgcttgttttaaagtgggctcagcacatagggttcccacgaagctccgaaactctaagtgtttgctgcaattttataaggacttcctgattggtttctcttctccccttccatttctgccttttgttcatttcatcctttcacttctttcccttcctccgtcctcctccttcctagttcatcccttctcttccaggcagccgcggtgcccaaccacacttgtcggctccagtccccagaactctgcctgccctttgtcctcctgctgccagtaccagccccaccctgttttgagccctgaggaggccttgggctctgctgagtccgacctggcctgtctgtgaagagcaagagagcagcaaggtcttgctctcctaggtagccccctcttccctggtaagaaaaagcaaaaggcatttcccaccctgaacaacgagccttttcacccttctactctagagaagtggactggaggagctgggcccgatttggtagttgaggaaagcacagaggcctcctgtggcctgccagtcatcgagtggcccaacaggggctccatgccagccgaccttgacctcactcagaagtccagagtctagcgtagtgcagcagggcagtagcggtaccaatgcagaactcccaagacccgagctgggaccagtacctgggtccccagcccttcctctgctcccccttttccctcggagttcttcttgaatggcaatgttttgcttttgctcgatgcagacagggggccagaacaccacacatttcactgtctgtctggtccatagctgtggtgtaggggcttagaggcatgggcttgctgtgggtttttaattgatcagttttcatgtgggatcccatctttttaacctctgttcaggaagtccttatctagctgcatatcttcatcatattggtatatccttttctgtgtttacagagatgtctcttatatctaaatctgtccaactgagaagtaccttatcaaagtagcaaatgagacagcagtcttatgcttccagaaacacccacaggcatgtcccatgtgagctgctgccatgaactgtcaagtgtgtgttgtcttgtgtatttcagttattgtccctggcttccttactatggtgtaatcatgaaggagtgaaacatcatagaaactgtctagcacttccttgccagtctttagtgatcaggaaccatagttgacagttccaatcagtagcttaagaaaaaaccgtgtttgtctcttctggaatggttagaagtgagggagtttgccccgttctgtttgtagagtctcatagttggactttctagcatatatgtgtccatttccttatgctgtaaaagcaagtcctgcaaccaaactcccatcagcccaatccctgatccctgatcccttccacctgctctgctgatgacccccccagcttcacttctgactcttccccaggaagggaaggggggtcagaagagagggtgagtcctccagaactcttcctccaaggacagaaggctcctgcccccatagtggcctcgaactcctggcactaccaaaggacacttatccacgagagcgcagcatccgaccaggttgtcactgagaagatgtttattttggtcagttgggtttttatgtattatacttagtcaaatgtaatgtggcttctggaatcattgtccagagctgcttccccgtcacctgggcgtcatctggtcctggtaagaggagtgcgtggcccaccaggcccccctgtcacccatgacagttcattcagggccgatggggcagtcgtggttgggaacacagcatttcaagcgtcactttatttcattcgggccccacctgcagctccctcaaagaggcagttgcccagcctctttcccttccagtttattccagagctgccagtggggcctgaggctccttagggttttctctctatttccccctttcttcctcattccctcgtctttcccaaaggcatcacgagtcagtcgcctttcagcaggcagccttggcggtttatcgccctggcaggcaggggccctgcagctctcatgctgcccctgccttggggtcaggttgacaggaggttggagggaaagccttaagctgcaggattctcaccagctgtgtccggcccagttttggggtgtgacctcaatttcaattttgtctgtacttgaacattatgaagatgggggcctctttcagtgaatttgtgaacagcagaattgaccgacagctttccagtacccatggggctaggtcattaaggccacatccacagtctcccccacccttgttccagttgttagttactacctcctctcctgacaatactgtatgtcgtcgagctccccccaggtctacccctcccggccctgcctgctggtgggcttgtcatagccagtgggattgccggtcttgacagctcagtgagctggagatacttggtcacagccaggcgctagcacagctcccttctgttgatgctgtattcccatatcaaaagacacaggggacacccagaaacgccacatcccccaatccatcagtgccaaactagccaacggccccagcttctcagctcgctggatggcggaagctgctactcgtgagcgccagtgcgggtgcagacaatcttctgttgggtggcatcattccaggcccgaagcatgaacagtgcacctgggacagggagcagccccaaattgtcacctgcttctctgcccagcttttcattgctgtgacagtgatggcgaaagagggtaataaccagacacaaactgccaagttgggtggagaaaggagtttctttagctgacagaatctctgaattttaaatcacttagtaagcggctcaagcccaggagggagcagagggatacgagcggagtcccctgcgcgggaccatctggaattggtttagcccaagtggagcctgacagccagaactctgtgtcccccgtctaaccacagctccttttccagagcattccagtcaggctctctgggctgactgggccaggggaggttacaggtaccagttctttaagaagatctttgggcatatacatttttagcctgtgtcattgccccaaatggattcctgtttcaagttcacacctgcagattctaggacctgtgtcctagacttcagggagtcagctgtttctagagttcctaccatggagtgggtctggaggacctgcccggtgggggggcagagccctgctccctccgggtcttcctactcttctctctgctctgacgggatttgttgattctctccattttggtgtctttctcttttagatattgtatcaatctttagaaaaggcatagtctacttgttataaatcgttaggatactgcctcccccagggtctaaaattacatattagaggggaaaagctgaacactgaagtcagttctcaacaatttagaaggaaaacctagaaaacatttggcagaaaattacatttcgatgtttttgaatgaatacgagcaagcttttacaacagtgctgatctaaaaatacttagcacttggcctgagatgcctggtgagcattacaggcaaggggaatctggaggtagccgacctgaggacatggcttctgaacctgtcttttgggagtggtatggaaggtggagcgttcaccagtgacctggaaggcccagcaccaccctccttcccactcttctcatcttgacagagcctgccccagcgctgacgtgtcaggaaaacacccagggaactaggaaggcacttctgcctgaggggcagcctgccttgcccactcctgctctgctcgcctcggatcagctgagccttctgagctggcctctcactgcctccccaaggccccctgcctgccctgtcaggaggcagaaggaagcaggtgtgagggcagtgcaaggagggagcacaacccccagctcccgctccgggctccgacttgtgcacaggcagagcccagaccctggaggaaatcctacctttgaattcaagaacatttggggaatttggaaatctctttgcccccaaacccccattctgtcctacctttaatcaggtcctgctcagcagtgagagcagatgaggtgaaaaggccaagaggtttggctcctgcccactgatagcccctctccccgcagtgtttgtgtgtcaagtggcaaagctgttcttcctggtgaccctgattatatccagtaacacatagactgtgcgcataggcctgctttgtctcctctatcctgggcttttgttttgctttttagttttgcttttagtttttctgtcccttttatttaacgcaccgactagacacacaaagcagttgaatttttatatatatatctgtatattgcacaattataaactcattttgcttgtggctccacacacacaaaaaaagacctgttaaaattatacctgttgcttaattacaatatttctgataaccatagcataggacaagggaaaataaaaaaagaaaaaaaagaaaaaaaaacgacaaatctgtctgctggtcacttcttctgtccaagcagattcgtggtcttttcctcgcttctttcaagggctttcctgtgccaggtgaaggaggctccaggcagcacccaggttttgcactcttgtttctcccgtgcttgtgaaagaggtcccaaggttctgggtgcaggagcgctcccttgacctgctgaagtccggaacgtagtcggcacagcctggtcgccttccacctctgggagctggagtccactggggtggcctgactcccccagtccccttcccgtgacctggtcagggtgagcccatgtggagtcagcctcgcaggcctccctgccagtagggtccgagtgtgtttcatccttcccactctgtcgagcctgggggctggagcggagacgggaggcctggcctgtctcggaacctgtgagctgcaccaggtagaacgccagggaccccagaatcatgtgcgtcagtccaaggggtcccctccaggagtagtgaagactccagaaatgtccctttcttctcccccatcctacgagtaattgcatttgcttttgtaattcttaatgagcaatatctgctagagagtttagctgtaacagttctttttgatcatctttttttaataattagaaacaccaaaaaaatccagaaacttgttcttccaaagcagagagcattataatcaccagggccaaaagcttccctccctgctgtcattgcttcttctgaggcctgaatccaaaagaaaaacagccataggccctttcagtggccgggctacccgtgagcccttcggaggaccagggctggggcagcctctgggcccacatccggggccagctccggcgtgtgttcagtgttagcagtgggtcatgatgctctttcccacccagcctgggataggggcagaggaggcgaggaggccgttgccgctgatgtttggccgtgaacaggtgggtgtctgcgtgcgtccacgtgcgtgttttctgactgacatgaaatcgacgcccgagttagcctcacccggtgacctctagccctgcccggatggagcggggcccacccggttcagtgtttctggggagctggacagtggagtgcaaaaggcttgcagaacttgaagcctgctccttcccttgctaccacggcctcctttccgtttgatttgtcactgcttcaatcaataacagccgctccagagtcagtagtcaatgaatatatgaccaaatatcaccaggactgttactcaatgtgtgccgagcccttgcccatgctgggctcccgtgtatctggacactgtaacgtgtgctgtgtttgctccccttccccttccttctttgccctttacttgtctttctggggtttttctgtttgggtttggtttggtttttatttctccttttgtgttccaaacatgaggttctctctactggtcctcttaactgtggtgttgaggcttatatttgtgtaatttttggtgggtgaaaggaattttgctaagtaaatctcttctgtgtttgaactgaagtctgtattgtaactatgtttaaagtaattgttccagagacaaatatttctagacactttttctttacaaacaaaagcattcggagggagggggatggtgactgagatgagaggggagagctgaacagatgacccctgcccagatcagccagaagccacccaaagcagtggagcccaggagtcccactccaagccagcaagccgaatagctgatgtgttgccactttccaagtcactgcaaaaccaggttttgttccgcccagtggattcttgttttgcttcccctccccccgagattattaccaccatcccgtgcttttaaggaaaggcaagattgatgtttccttgaggggagccaggaggggatgtgtgtgtgcagagctgaagagctggggagaatggggctgggcccacccaagcaggaggctgggacgctctgctgtgggcacaggtcaggctaatgttggcagatgcagctcttcctggacaggccaggtggtgggcattctctctccaaggtgtgccccgtgggcattactgtttaagacacttccgtcacatcccaccccatcctccagggctcaacactgtgacatctctattccccaccctccccttcccagggcaataaaatgaccatggagggggcttgcactctcttggctgtcacccgatcgccagcaaaacttagatgtgagaaaaccccttcccattccatggcgaaaacatctccttagaaaagccattaccctcattaggcatggttttgggctcccaaaacacctgacagcccctccctcctctgagaggcggagagtgctgactgtagtgaccattgcatgccgggtgcagcatctggaagagctaggcagggtgtctgccccctcctgagttgaagtcatgctcccctgtgccagcccagaggccgagagctatggacagcattgccagtaacacaggccaccctgtgcagaagggagctggctccagcctggaaacctgtctgaggttgggagaggtgcacttggggcacagggagaggccgggacacacttagctggagatgtctctaaaagccctgtatcgtattcaccttcagtttttgtgttttgggacaattactttagaaaataagtaggtcgttttaaaaacaaaaattattgattgcttttttgtagtgttcagaaaaaaggttctttgtgtatagccaaatgactgaaagcactgatatatttaaaaacaaaaggcaatttattaaggaaatttgtaccatttcagtaaacctgtctgaatgtacctgtatacgtttcaaaaacaccccccccccactgaatccctgtaacctatttattatataaagagtttgccttataaattt

SEQ ID NO: 3 - DNA, 20 bp, Artificial sequence
  Primer
tatttgatcaatccccaggg

SEQ ID NO: 4 - DNA, 20 bp, Artificial sequence
  Primer
ctccctctcccagttaccgt

SEQ ID NO: 5 - DNA, 22 bp, Artificial sequence
  Primer
aggagagactggaagaaaagtc

SEQ ID NO: 6 - DNA, 20 bp, Artificial sequence
  Primer
cttgaggggtttgtccttga

SEQ ID NO: 7 - DNA, 23 bp, Artificial sequence
  Primer
ctcaccagttcctgctttgatgt

SEQ ID NO: 8 - DNA, 22 bp, Artificial sequence
  Primer
aggagagactggaggaaaagtc

SEQ ID NO: 9 - DNA, 25 bp, Artificial sequence
  Primer
cttaaacttcagtggcttgtctctg

SEQ ID NO: 10 - DNA, 21 bp, Artificial sequence
  Primer
cgggggacataaaagttattg

SEQ ID NO: 11 - DNA, 22 bp, Artificial sequence
  Primer
tgcattgttttaccagtgtcaa

SEQ ID NO: 12 - DNA, 25 bp, Artificial sequence
  Primer
tgaaggagtcttctatccgatctgt

SEQ ID NO: 13 - DNA, 21 bp, Artificial sequence
  Primer
cacttccttgacctcgatgct

SEQ ID NO: 14 - DNA, 26 bp, Artificial sequence
  Probe
agaccgtactccccatcaagaagcgc

SEQ ID NO: 15 - DNA, 20 bp, Artificial sequence
  Synthetic oligonucleotide
gtgcgcgcgagcccgaaatc

SEQ ID NO: 16 - DNA, 20 bp, Artificial sequence
  Synthetic oligonucleotide
ctctccgagaggagggagcg

SEQ ID NO: 17 - DNA, 20 bp, Artificial sequence
  Synthetic oligonucleotide
gccattttccggacggcttt

SEQ ID NO: 18 - DNA, 20 bp, Artificial sequence
  Synthetic oligonucleotide
tctctcctcctcgcctcctc

SEQ ID NO: 19 - DNA, 20 bp, Artificial sequence
  Synthetic oligonucleotide
acccccgccccccggcaagg

SEQ ID NO: 20 - DNA, 20 bp, Artificial sequence
  Synthetic oligonucleotide
agagacctcaacttgtcacg

SEQ ID NO: 21 - DNA, 20 bp, Artificial sequence
  Synthetic oligonucleotide
cattaagataaccatcattt

SEQ ID NO: 22 - DNA, 20 bp, Artificial sequence
  Synthetic oligonucleotide
ggaactggtgagtctgtatt

SEQ ID NO: 23 - DNA, 20 bp, Artificial sequence
  Synthetic oligonucleotide
gaagcaaggtgtattctggg

SEQ ID NO: 24 - DNA, 20 bp, Artificial sequence
  Synthetic oligonucleotide
ctaccatggaatcctgttgg

SEQ ID NO: 25 - DNA, 20 bp, Artificial sequence
  Synthetic oligonucleotide
ttttctataaatccatgtat

SEQ ID NO: 26 - DNA, 20 bp, Artificial sequence
  Synthetic oligonucleotide
tagccccactcccggataag

SEQ ID NO: 27 - DNA, 20 bp, Artificial sequence
  Synthetic oligonucleotide
actcaagcccaaggagttca

SEQ ID NO: 28 - DNA, 20 bp, Artificial sequence
  Synthetic oligonucleotide
gctttaatgctttattttta

SEQ ID NO: 29 - DNA, 20 bp, Artificial sequence
  Synthetic oligonucleotide
tgccaacagcaggcccagcg

SEQ ID NO: 30 - DNA, 20 bp, Artificial sequence
  Synthetic oligonucleotide
gatatcagtgaggaagttgt

SEQ ID NO: 31 - DNA, 20 bp, Artificial sequence
  Synthetic oligonucleotide
cgtgccatggaagtccttcc

SEQ ID NO: 32 - DNA, 20 bp, Artificial sequence
  Synthetic oligonucleotide
ggtgagctgatgctatatga

SEQ ID NO: 33 - DNA, 20 bp, Artificial sequence
  Synthetic oligonucleotide
aggcggcagtggcttacgcc

SEQ ID NO: 34 - DNA, 20 bp, Artificial sequence
  Synthetic oligonucleotide
agccccttaattttgttctc

SEQ ID NO: 35 - DNA, 20 bp, Artificial sequence
  Synthetic oligonucleotide
tggcggctcaagaaccagcc

SEQ ID NO: 36 - DNA, 20 bp, Artificial sequence
  Synthetic oligonucleotide
caaatattagaatagactca

SEQ ID NO: 37 - DNA, 20 bp, Artificial sequence
  Synthetic oligonucleotide
tgggactcagattctatagg

SEQ ID NO: 38 - DNA, 20 bp, Artificial sequence
  Synthetic oligonucleotide
gtcctggaacgacaggcttg

SEQ ID NO: 39 - DNA, 20 bp, Artificial sequence
  Synthetic oligonucleotide
ccaaatttataacttaagaa

SEQ ID NO: 40 - DNA, 20 bp, Artificial sequence
  Synthetic oligonucleotide
ggtgatgtgtattttactac

SEQ ID NO: 41 - DNA, 20 bp, Artificial sequence
  Synthetic oligonucleotide
tggtgggacaaaaattgtgg

SEQ ID NO: 42 - DNA, 20 bp, Artificial sequence
  Synthetic oligonucleotide
aaataagcatctggcatttg

SEQ ID NO: 43 - DNA, 20 bp, Artificial sequence
  Synthetic oligonucleotide
tacattgaaaaacagccaga

SEQ ID NO: 44 - DNA, 20 bp, Artificial sequence
  Synthetic oligonucleotide
ggatccatgcgagagaagca

SEQ ID NO: 45 - DNA, 20 bp, Artificial sequence
  Synthetic oligonucleotide
tataatatcattcagcctca

SEQ ID NO: 46 - DNA, 20 bp, Artificial sequence
  Synthetic oligonucleotide
cagcaggaagagtccagaga

SEQ ID NO: 47 - DNA, 20 bp, Artificial sequence
  Synthetic oligonucleotide
agaaacctgccaggtgtggt

SEQ ID NO: 48 - DNA, 20 bp, Artificial sequence
  Synthetic oligonucleotide
ccaggtgtggcccagggtgg

SEQ ID NO: 49 - DNA, 20 bp, Artificial sequence
  Synthetic oligonucleotide
ggcatcctacaacccacaga

SEQ ID NO: 50 - DNA, 20 bp, Artificial sequence
  Synthetic oligonucleotide
tgacttttcttccctgagcc

SEQ ID NO: 51 - DNA, 20 bp, Artificial sequence
  Synthetic oligonucleotide
gggtttgtccttgaggccct

SEQ ID NO: 52 - DNA, 20 bp, Artificial sequence
  Synthetic oligonucleotide
ctcttctttcttatctttct

SEQ ID NO: 53 - DNA, 20 bp, Artificial sequence
  Synthetic oligonucleotide
cttgccctctttctcttctt

SEQ ID NO: 54 - DNA, 20 bp, Artificial sequence
  Synthetic oligonucleotide
tggctgcacgggctcatgct

SEQ ID NO: 55 - DNA, 20 bp, Artificial sequence
  Synthetic oligonucleotide
gtggtgggctgatggctgca

SEQ ID NO: 56 - DNA, 20 bp, Artificial sequence
  Synthetic oligonucleotide
ctgctttgcctgcctctgcg

SEQ ID NO: 57 - DNA, 20 bp, Artificial sequence
  Synthetic oligonucleotide
aagcttccggcacagccggg

SEQ ID NO: 58 - DNA, 20 bp, Artificial sequence
  Synthetic oligonucleotide
ggtcacggatgatggagcgc

SEQ ID NO: 59 - DNA, 20 bp, Artificial sequence
  Synthetic oligonucleotide
ttccgtgtccagccttcagg

SEQ ID NO: 60 - DNA, 20 bp, Artificial sequence
  Synthetic oligonucleotide
cagcagagcggccagatttc

SEQ ID NO: 61 - DNA, 20 bp, Artificial sequence
  Synthetic oligonucleotide
tgtccctgccctccctgccc

SEQ ID NO: 62 - DNA, 20 bp, Artificial sequence
  Synthetic oligonucleotide
gcgaaaggcttttccctggg

SEQ ID NO: 63 - DNA, 20 bp, Artificial sequence
  Synthetic oligonucleotide
gaagtacgcaatcaactcca

SEQ ID NO: 64 - DNA, 20 bp, Artificial sequence
  Synthetic oligonucleotide
gggatgtgtcgcctaccttt

SEQ ID NO: 65 - DNA, 20 bp, Artificial sequence
  Synthetic oligonucleotide
cgtgaagtcaaaatcattag

SEQ ID NO: 66 - DNA, 20 bp, Artificial sequence
  Synthetic oligonucleotide
ttaggtggtttctgctctcg

SEQ ID NO: 67 - DNA, 20 bp, Artificial sequence
  Synthetic oligonucleotide
cggcctctgccagttcctgg

SEQ ID NO: 68 - DNA, 20 bp, Artificial sequence
  Synthetic oligonucleotide
acccttttcacctgcacacc

SEQ ID NO: 69 - DNA, 20 bp, Artificial sequence
  Synthetic oligonucleotide
aaggagcttcccaggacttt

SEQ ID NO: 70 - DNA, 20 bp, Artificial sequence
  Synthetic oligonucleotide
tggcgaagtttgaaaaggca

SEQ ID NO: 71 - DNA, 20 bp, Artificial sequence
  Synthetic oligonucleotide
agccttgccccctggcgaag

SEQ ID NO: 72 - DNA, 20 bp, Artificial sequence
  Synthetic oligonucleotide
tggatgtggtggccccaccc

SEQ ID NO: 73 - DNA, 20 bp, Artificial sequence
  Synthetic oligonucleotide
gcttttcgcttcctgccggg

SEQ ID NO: 74 - DNA, 20 bp, Artificial sequence
  Synthetic oligonucleotide
gtttcttgggaatggcctga

SEQ ID NO: 75 - DNA, 20 bp, Artificial sequence
  Synthetic oligonucleotide
ggctgccaccacactccccg

SEQ ID NO: 76 - DNA, 20 bp, Artificial sequence
  Synthetic oligonucleotide
ttcacggctttctttttggc

SEQ ID NO: 77 - DNA, 20 bp, Artificial sequence
  Synthetic oligonucleotide
ctcctgcacagatcggatag

SEQ ID NO: 78 - DNA, 20 bp, Artificial sequence
  Synthetic oligonucleotide
tctcccgggtcttgcgcttc

SEQ ID NO: 79 - DNA, 20 bp, Artificial sequence
  Synthetic oligonucleotide
cttcaccacttccttgacct

SEQ ID NO: 80 - DNA, 20 bp, Artificial sequence
  Synthetic oligonucleotide
tcagtcctttcccgctcttc

SEQ ID NO: 81 - DNA, 20 bp, Artificial sequence
  Synthetic oligonucleotide
cttgcttttccgcccagggc

SEQ ID NO: 82 - DNA, 20 bp, Artificial sequence
  Synthetic oligonucleotide
ggtgatggtggtggtgctcc

SEQ ID NO: 83 - DNA, 20 bp, Artificial sequence
  Synthetic oligonucleotide
gctgctgctcaagtcctggg

SEQ ID NO: 84 - DNA, 20 bp, Artificial sequence
  Synthetic oligonucleotide
ctccagtgagcctcctctgg

SEQ ID NO: 85 - DNA, 20 bp, Artificial sequence
  Synthetic oligonucleotide
aaccgcgggctgagtcttag

SEQ ID NO: 86 - DNA, 20 bp, Artificial sequence
  Synthetic oligonucleotide
tggcggcggtggcaaccgcg

SEQ ID NO: 87 - DNA, 20 bp, Artificial sequence
  Synthetic oligonucleotide
ttttctgcggccgtggcggc

SEQ ID NO: 88 - DNA, 20 bp, Artificial sequence
  Synthetic oligonucleotide
ctctccctcccctcggtgtt

SEQ ID NO: 89 - DNA, 20 bp, Artificial sequence
  Synthetic oligonucleotide
cttggcatggaggatgaaac

SEQ ID NO: 90 - DNA, 20 bp, Artificial sequence
  Synthetic oligonucleotide
tccggctgtccacaggctcc

SEQ ID NO: 91 - DNA, 20 bp, Artificial sequence
  Synthetic oligonucleotide
aatccgctccgtgtaaagtc

SEQ ID NO: 92 - DNA, 20 bp, Artificial sequence
  Synthetic oligonucleotide
cagctgcctttattcttgtt

SEQ ID NO: 93 - DNA, 20 bp, Artificial sequence
  Synthetic oligonucleotide
gtcagagccctacccataag

SEQ ID NO: 94 - DNA, 20 bp, Artificial sequence
  Synthetic oligonucleotide
agcgcgcgcgccgccgacgc

SEQ ID NO: 95 - DNA, 20 bp, Artificial sequence
  Synthetic oligonucleotide
cttttaccacagccctctct

SEQ ID NO: 96 - DNA, 20 bp, Artificial sequence
  Synthetic oligonucleotide
ccgctcggcgcggcggcggc

SEQ ID NO: 97 - DNA, 20 bp, Artificial sequence
  Synthetic oligonucleotide
tcagtttgggtgattcggtc

SEQ ID NO: 98 - DNA, 20 bp, Artificial sequence
  Synthetic oligonucleotide
cagcacagcgggaacacatt

SEQ ID NO: 99 - DNA, 20 bp, Artificial sequence
  Synthetic oligonucleotide
tatttttatggagcagtctc

SEQ ID NO: 100 - DNA, 20 bp, Artificial sequence
  Synthetic oligonucleotide
atgtcacatcaaagcaggaa

SEQ ID NO: 101 - DNA, 20 bp, Artificial sequence
  Synthetic oligonucleotide
ttggagctggtctacagaag

SEQ ID NO: 102 - DNA, 20 bp, Artificial sequence
  Synthetic oligonucleotide
agccctaacatcccagctac

SEQ ID NO: 103 - DNA, 20 bp, Artificial sequence
  Synthetic oligonucleotide
cacactgacctttcagggct

SEQ ID NO: 104 - DNA, 20 bp, Artificial sequence
  Synthetic oligonucleotide
taaaaaaggatttcctaagt

SEQ ID NO: 105 - DNA, 20 bp, Artificial sequence
  Synthetic oligonucleotide
gtacacacacgctttttttt

SEQ ID NO: 106 - DNA, 20 bp, Artificial sequence
  Synthetic oligonucleotide
gaaagccgagcctggccggg

SEQ ID NO: 107 - DNA, 20 bp, Artificial sequence
  Synthetic oligonucleotide
gaagaaaatgtggatttttt

SEQ ID NO: 108 - DNA, 20 bp, Artificial sequence
  Synthetic oligonucleotide
cgagaatgagactccgtatc

SEQ ID NO: 109 - DNA, 20 bp, Artificial sequence
  Synthetic oligonucleotide
aaacccaaaccaccttaccc

SEQ ID NO: 110 - DNA, 20 bp, Artificial sequence
  Synthetic oligonucleotide
aaaataaagtcaggaggctg

SEQ ID NO: 111 - DNA, 20 bp, Artificial sequence
  Synthetic oligonucleotide
aaaaatggagggcacagtgg

SEQ ID NO: 112 - DNA, 20 bp, Artificial sequence
  Synthetic oligonucleotide
ggtttttctcctttattatc

SEQ ID NO: 113 - DNA, 20 bp, Artificial sequence
  Synthetic oligonucleotide
tatgttggcctagaactcct

SEQ ID NO: 114 - DNA, 20 bp, Artificial sequence
  Synthetic oligonucleotide
tgctctcatattcacccacg

SEQ ID NO: 115 - DNA, 20 bp, Artificial sequence
  Synthetic oligonucleotide
gtgcagagactcaagggagg

SEQ ID NO: 116 - DNA, 20 bp, Artificial sequence
  Synthetic oligonucleotide
gctaagcctcctggtgaacc

SEQ ID NO: 117 - DNA, 20 bp, Artificial sequence
  Synthetic oligonucleotide
gtatgaacatcagctgacgc

SEQ ID NO: 118 - DNA, 20 bp, Artificial sequence
  Synthetic oligonucleotide
aggcgcgctggtgcaagcct

SEQ ID NO: 119 - DNA, 20 bp, Artificial sequence
  Synthetic oligonucleotide
cagccactctttttttttga

SEQ ID NO: 120 - DNA, 20 bp, Artificial sequence
  Synthetic oligonucleotide
gtacctgggaggaactacaa

SEQ ID NO: 121 - DNA, 20 bp, Artificial sequence
  Synthetic oligonucleotide
agggcgagagatccaggact

SEQ ID NO: 122 - DNA, 20 bp, Artificial sequence
  Synthetic oligonucleotide
ggattagggaattagatgca

SEQ ID NO: 123 - DNA, 20 bp, Artificial sequence
  Synthetic oligonucleotide
ggaaagcctgtcttttaaaa

SEQ ID NO: 124 - DNA, 20 bp, Artificial sequence
  Synthetic oligonucleotide
ccagatggtgtttccaattc

SEQ ID NO: 125 - DNA, 20 bp, Artificial sequence
  Synthetic oligonucleotide
acttctagaccgggcgcagt

SEQ ID NO: 126 - DNA, 20 bp, Artificial sequence
  Synthetic oligonucleotide
gtacaatgaatgaacttttt

SEQ ID NO: 127 - DNA, 20 bp, Artificial sequence
  Synthetic oligonucleotide
caaacatatctactgcattc

SEQ ID NO: 128 - DNA, 20 bp, Artificial sequence
  Synthetic oligonucleotide
acaggtaaccccatctaggc

SEQ ID NO: 129 - DNA, 20 bp, Artificial sequence
  Synthetic oligonucleotide
ggaggtcctggtcttctgac

SEQ ID NO: 130 - DNA, 20 bp, Artificial sequence
  Synthetic oligonucleotide
ttatctttcttcaccttttt

SEQ ID NO: 131 - DNA, 20 bp, Artificial sequence
  Synthetic oligonucleotide
ctctttctcttctttcttat

SEQ ID NO: 132 - DNA, 20 bp, Artificial sequence
  Synthetic oligonucleotide
cacgggctcatgcttgccct

SEQ ID NO: 133 - DNA, 20 bp, Artificial sequence
  Synthetic oligonucleotide
ggctgatggctgcacgggct

SEQ ID NO: 134 - DNA, 20 bp, Artificial sequence
  Synthetic oligonucleotide
tgcgggctcagcagagtggt

SEQ ID NO: 135 - DNA, 20 bp, Artificial sequence
  Synthetic oligonucleotide
gacccttctgatgtctctgc

SEQ ID NO: 136 - DNA, 20 bp, Artificial sequence
  Synthetic oligonucleotide
aggcagaagcttccggcaca

SEQ ID NO: 137 - DNA, 20 bp, Artificial sequence
  Synthetic oligonucleotide
tcatacatgggtccccggtc

SEQ ID NO: 138 - DNA, 20 bp, Artificial sequence
  Synthetic oligonucleotide
tttcctttgcttaagcttcc

SEQ ID NO: 139 - DNA, 20 bp, Artificial sequence
  Synthetic oligonucleotide
tacacatcatacttcccagc

SEQ ID NO: 140 - DNA, 20 bp, Artificial sequence
  Synthetic oligonucleotide
tcaactccactttagagcga

SEQ ID NO: 141 - DNA, 20 bp, Artificial sequence
  Synthetic oligonucleotide
gcctaccttttcgaagtacg

SEQ ID NO: 142 - DNA, 20 bp, Artificial sequence
  Synthetic oligonucleotide
ggtccagggatgtgtcgcct

SEQ ID NO: 143 - DNA, 20 bp, Artificial sequence
  Synthetic oligonucleotide
tccctctcccagttaccgtg

SEQ ID NO: 144 - DNA, 20 bp, Artificial sequence
  Synthetic oligonucleotide
tggagctttgggagatttgg

SEQ ID NO: 145 - DNA, 20 bp, Artificial sequence
  Synthetic oligonucleotide
cgtggccgccttgggtctcg

SEQ ID NO: 146 - DNA, 20 bp, Artificial sequence
  Synthetic oligonucleotide
aggacttttctccaggaccc

SEQ ID NO: 147 - DNA, 20 bp, Artificial sequence
  Synthetic oligonucleotide
aggcatcttgacaaggagct

SEQ ID NO: 148 - DNA, 20 bp, Artificial sequence
  Synthetic oligonucleotide
gccccctggcgaagtttgaa

SEQ ID NO: 149 - DNA, 20 bp, Artificial sequence
  Synthetic oligonucleotide
ccccacccccctcagccttg

SEQ ID NO: 150 - DNA, 20 bp, Artificial sequence
  Synthetic oligonucleotide
ccatgacctgggtggatgtg

SEQ ID NO: 151 - DNA, 20 bp, Artificial sequence
  Synthetic oligonucleotide
ctgagggtcggcctcagctt

SEQ ID NO: 152 - DNA, 20 bp, Artificial sequence
  Synthetic oligonucleotide
cccggctttcggccccgttt

SEQ ID NO: 153 - DNA, 20 bp, Artificial sequence
  Synthetic oligonucleotide
tggcctcggcggcagcggct

SEQ ID NO: 154 - DNA, 20 bp, Artificial sequence
  Synthetic oligonucleotide
tcggatagaagactccttca

SEQ ID NO: 155 - DNA, 20 bp, Artificial sequence
  Synthetic oligonucleotide
tacggtctcctgcacagatc

SEQ ID NO: 156 - DNA, 20 bp, Artificial sequence
  Synthetic oligonucleotide
acctcgatgctgaccgtctc

SEQ ID NO: 157 - DNA, 20 bp, Artificial sequence
  Synthetic oligonucleotide
cttctcaccgagggtggaca

SEQ ID NO: 158 - DNA, 20 bp, Artificial sequence
  Synthetic oligonucleotide
gggctcttacaggtcttcag

SEQ ID NO: 159 - DNA, 20 bp, Artificial sequence
  Synthetic oligonucleotide
ctgctgctgcgccccttggg

SEQ ID NO: 160 - DNA, 20 bp, Artificial sequence
  Synthetic oligonucleotide
tcgggctcaggtggaggtgg

SEQ ID NO: 161 - DNA, 20 bp, Artificial sequence
  Synthetic oligonucleotide
ctgggcatcttctcctcttt

SEQ ID NO: 162 - DNA, 20 bp, Artificial sequence
  Synthetic oligonucleotide
gtcttagctggctccttggg

SEQ ID NO: 163 - DNA, 20 bp, Artificial sequence
  Synthetic oligonucleotide
ggtggcaaccgcgggctgag

SEQ ID NO: 164 - DNA, 20 bp, Artificial sequence
  Synthetic oligonucleotide
cggccgtggcggcggtggca

SEQ ID NO: 165 - DNA, 20 bp, Artificial sequence
  Synthetic oligonucleotide
tgtttgtacttttctgcggc

SEQ ID NO: 166 - DNA, 20 bp, Artificial sequence
  Synthetic oligonucleotide
aaacaatgtctttgcgctct

SEQ ID NO: 167 - DNA, 20 bp, Artificial sequence
  Synthetic oligonucleotide
ctcctctctgtttggccttg

SEQ ID NO: 168 - DNA, 20 bp, Artificial sequence
  Synthetic oligonucleotide
agtcagctaactctctcggt

SEQ ID NO: 169 - DNA, 20 bp, Artificial sequence
  Synthetic oligonucleotide
tgttggtttgctttgcaatc

SEQ ID NO: 170 - DNA, 20 bp, Artificial sequence
  Synthetic oligonucleotide
taaggagaagagacaacagc

SEQ ID NO: 171 - DNA, 20 bp, Artificial sequence
  Synthetic oligonucleotide
ttaatcgggaagctttgtca

SEQ ID NO: 172 - DNA, 20 bp, Artificial sequence
  Synthetic oligonucleotide
gaggagggagcgcgcgcgcc

SEQ ID NO: 173 - DNA, 20 bp, Artificial sequence
  Synthetic oligonucleotide
ccggacggcttttaccacag

SEQ ID NO: 174 - DNA, 20 bp, Artificial sequence
  Synthetic oligonucleotide
ctcctcctccgctcggcgcg

SEQ ID NO: 175 - DNA, 20 bp, Artificial sequence
  Synthetic oligonucleotide
atgcttcatttttacagtat

SEQ ID NO: 176 - DNA, 20 bp, Artificial sequence
  Synthetic oligonucleotide
gagccagaggctgggtgcgg

SEQ ID NO: 177 - DNA, 20 bp, Artificial sequence
  Synthetic oligonucleotide
tgagtctgtatttttatgga

SEQ ID NO: 178 - DNA, 20 bp, Artificial sequence
  Synthetic oligonucleotide
ggagtcacatgtcacatcaa

SEQ ID NO: 179 - DNA, 20 bp, Artificial sequence
  Synthetic oligonucleotide
gaatcctgttggagctggtc

SEQ ID NO: 180 - DNA, 20 bp, Artificial sequence
  Synthetic oligonucleotide
cttccctgagccctaacatc

SEQ ID NO: 181 - DNA, 20 bp, Artificial sequence
  Synthetic oligonucleotide
cccacagcagtaaaagagaa

SEQ ID NO: 182 - DNA, 20 bp, Artificial sequence
  Synthetic oligonucleotide
accccagtagttgagattac

SEQ ID NO: 183 - DNA, 20 bp, Artificial sequence
  Synthetic oligonucleotide
atagtagttgccagagggtg

SEQ ID NO: 184 - DNA, 20 bp, Artificial sequence
  Synthetic oligonucleotide
ggcttctattgtaaaactat

SEQ ID NO: 185 - DNA, 20 bp, Artificial sequence
  Synthetic oligonucleotide
actggtttttaagagatggg

SEQ ID NO: 186 - DNA, 20 bp, Artificial sequence
  Synthetic oligonucleotide
taaaatctatgggaataaaa

SEQ ID NO: 187 - DNA, 20 bp, Artificial sequence
  Synthetic oligonucleotide
gaaatgtgggcttggcatgg

SEQ ID NO: 188 - DNA, 20 bp, Artificial sequence
  Synthetic oligonucleotide
aacatggtttagtagaaacc

SEQ ID NO: 189 - DNA, 20 bp, Artificial sequence
  Synthetic oligonucleotide
ggtattataattttgtaatt

SEQ ID NO: 190 - DNA, 20 bp, Artificial sequence
  Synthetic oligonucleotide
caacattccatttatttagg

SEQ ID NO: 191 - DNA, 20 bp, Artificial sequence
  Synthetic oligonucleotide
attttcaccctttaaaaatc

SEQ ID NO: 192 - DNA, 20 bp, Artificial sequence
  Synthetic oligonucleotide
taatacagtgacaagcatcc

SEQ ID NO: 193 - DNA, 20 bp, Artificial sequence
  Synthetic oligonucleotide
tccatcttgcaggtggagta

SEQ ID NO: 194 - DNA, 20 bp, Artificial sequence
  Synthetic oligonucleotide
gaagccaaaaaagcaacaaa

SEQ ID NO: 195 - DNA, 20 bp, Artificial sequence
  Synthetic oligonucleotide
ccaagacaaggaaaaacggg

SEQ ID NO: 196 - DNA, 20 bp, Artificial sequence
  Synthetic oligonucleotide
ctagctatcagctgggcatg

SEQ ID NO: 197 - DNA, 20 bp, Artificial sequence
  Synthetic oligonucleotide
tgccttgttgggtagtacag

SEQ ID NO: 198 - DNA, 20 bp, Artificial sequence
  Synthetic oligonucleotide
gctaagttagaactccgtgg

SEQ ID NO: 199 - DNA, 20 bp, Artificial sequence
  Synthetic oligonucleotide
acacgcctgtaatcctgcat

SEQ ID NO: 200 - DNA, 20 bp, Artificial sequence
  Synthetic oligonucleotide
caactggaggccgggcgcga

SEQ ID NO: 201 - DNA, 20 bp, Artificial sequence
  Synthetic oligonucleotide
agcccacacagctgtctcag

SEQ ID NO: 202 - DNA, 20 bp, Artificial sequence
  Synthetic oligonucleotide
ttcctcatgaatgtgacctg

SEQ ID NO: 203 - DNA, 20 bp, Artificial sequence
  Synthetic oligonucleotide
gaggaacttgtctgagatca

SEQ ID NO: 204 - DNA, 20 bp, Artificial sequence
  Synthetic oligonucleotide
cagctactcgctagaaaggg

SEQ ID NO: 205 - DNA, 20 bp, Artificial sequence
  Synthetic oligonucleotide
ctccccataaaggagggagg

SEQ ID NO: 206 - DNA, 20 bp, Artificial sequence
  Synthetic oligonucleotide
ccatcatacactcagatctt

SEQ ID NO: 207 - DNA, 20 bp, Artificial sequence
  Synthetic oligonucleotide
ttgaggccctggaggtcctg

SEQ ID NO: 208 - DNA, 20 bp, Artificial sequence
  Synthetic oligonucleotide
ttctttcttatctttcttca

SEQ ID NO: 209 - DNA, 20 bp, Artificial sequence
  Synthetic oligonucleotide
gccctctttctcttctttct

SEQ ID NO: 210 - DNA, 20 bp, Artificial sequence
  Synthetic oligonucleotide
ctgcacgggctcatgcttgc

SEQ ID NO: 211 - DNA, 20 bp, Artificial sequence
  Synthetic oligonucleotide
gtgggctgatggctgcacgg

SEQ ID NO: 212 - DNA, 20 bp, Artificial sequence
  Synthetic oligonucleotide
cctgcctctgcgggctcagc

SEQ ID NO: 213 - DNA, 20 bp, Artificial sequence
  Synthetic oligonucleotide
cggagcctgacccttctgat

SEQ ID NO: 214 - DNA, 20 bp, Artificial sequence
  Synthetic oligonucleotide
gggaggcagaagcttccggc

SEQ ID NO: 215 - DNA, 20 bp, Artificial sequence
  Synthetic oligonucleotide
ccagccttcaggcagggtgg

SEQ ID NO: 216 - DNA, 20 bp, Artificial sequence
  Synthetic oligonucleotide
cggccagatttcctttgctt

SEQ ID NO: 217 - DNA, 20 bp, Artificial sequence
  Synthetic oligonucleotide
tgatcaaatacacatcatac

SEQ ID NO: 218 - DNA, 20 bp, Artificial sequence
  Synthetic oligonucleotide
gtacgcaatcaactccactt

SEQ ID NO: 219 - DNA, 20 bp, Artificial sequence
  Synthetic oligonucleotide
tgtgtcgcctaccttttcga

SEQ ID NO: 220 - DNA, 20 bp, Artificial sequence
  Synthetic oligonucleotide
caaaatcattagggtccagg

SEQ ID NO: 221 - DNA, 20 bp, Artificial sequence
  Synthetic oligonucleotide
tttctgctctcgccgggagg

SEQ ID NO: 222 - DNA, 20 bp, Artificial sequence
  Synthetic oligonucleotide
ccagttcctggagctttggg

SEQ ID NO: 223 - DNA, 20 bp, Artificial sequence
  Synthetic oligonucleotide
cacctgcacaccctctgacg

SEQ ID NO: 224 - DNA, 20 bp, Artificial sequence
  Synthetic oligonucleotide
gagcttcccaggacttttct

SEQ ID NO: 225 - DNA, 20 bp, Artificial sequence
  Synthetic oligonucleotide
gtttgaaaaggcatcttgac

SEQ ID NO: 226 - DNA, 20 bp, Artificial sequence
  Synthetic oligonucleotide
cttgccccctggcgaagttt

SEQ ID NO: 227 - DNA, 20 bp, Artificial sequence
  Synthetic oligonucleotide
tgtggtggccccacccccct

SEQ ID NO: 228 - DNA, 20 bp, Artificial sequence
  Synthetic oligonucleotide
tttgatcaccatgacctggg

SEQ ID NO: 229 - DNA, 20 bp, Artificial sequence
  Synthetic oligonucleotide
ggaatggcctgagggtcggc

SEQ ID NO: 230 - DNA, 20 bp, Artificial sequence
  Synthetic oligonucleotide
ccacactccccggctttcgg

SEQ ID NO: 231 - DNA, 20 bp, Artificial sequence
  Synthetic oligonucleotide
tttctttttggcctcggcgg

SEQ ID NO: 232 - DNA, 20 bp, Artificial sequence
  Synthetic oligonucleotide
ctgcacagatcggatagaag

SEQ ID NO: 233 - DNA, 20 bp, Artificial sequence
  Synthetic oligonucleotide
gtcttgcgcttcttgatggg

SEQ ID NO: 234 - DNA, 20 bp, Artificial sequence
  Synthetic oligonucleotide
cttccttgacctcgatgctg

SEQ ID NO: 235 - DNA, 20 bp, Artificial sequence
  Synthetic oligonucleotide
ttcccgctcttctcaccgag

SEQ ID NO: 236 - DNA, 20 bp, Artificial sequence
  Synthetic oligonucleotide
tccgcccagggctcttacag

SEQ ID NO: 237 - DNA, 20 bp, Artificial sequence
  Synthetic oligonucleotide
tggtggtgctccttcttggg

SEQ ID NO: 238 - DNA, 20 bp, Artificial sequence
  Synthetic oligonucleotide
cggagctctcgggctcaggt

SEQ ID NO: 239 - DNA, 20 bp, Artificial sequence
  Synthetic oligonucleotide
agcctcctctgggcatcttc

SEQ ID NO: 240 - DNA, 20 bp, Artificial sequence
  Synthetic oligonucleotide
cgggctgagtcttagctggc

SEQ ID NO: 241 - DNA, 20 bp, Artificial sequence
  Synthetic oligonucleotide
ggcggtggcaaccgcgggct

SEQ ID NO: 242 - DNA, 20 bp, Artificial sequence
  Synthetic oligonucleotide
tctgcggccgtggcggcggt

SEQ ID NO: 243 - DNA, 20 bp, Artificial sequence
  Synthetic oligonucleotide
cccctcggtgtttgtacttt

SEQ ID NO: 244 - DNA, 20 bp, Artificial sequence
  Synthetic oligonucleotide
ggaggatgaaacaatgtctt

SEQ ID NO: 245 - DNA, 20 bp, Artificial sequence
  Synthetic oligonucleotide
tccacaggctcctctctgtt

SEQ ID NO: 246 - DNA, 20 bp, Artificial sequence
  Synthetic oligonucleotide
ccgtgtaaagtcagctaact

SEQ ID NO: 247 - DNA, 20 bp, Artificial sequence
  Synthetic oligonucleotide
tttattcttgttggtttgct

SEQ ID NO: 248 - DNA, 20 bp, Artificial sequence
  Synthetic oligonucleotide
cctacccataaggagaagag

SEQ ID NO: 249 - DNA, 20 bp, Artificial sequence
  Synthetic oligonucleotide
tatttcagttaatcgggaag

SEQ ID NO: 250 - DNA, 20 bp, Artificial sequence
  Synthetic oligonucleotide
acagccctctctccgagagg

SEQ ID NO: 251 - DNA, 20 bp, Artificial sequence
  Synthetic oligonucleotide
cggcggcggccattttccgg

SEQ ID NO: 252 - DNA, 20 bp, Artificial sequence
  Synthetic oligonucleotide
tggagcagtctctcctcctc

SEQ ID NO: 253 - DNA, 20 bp, Artificial sequence
  Synthetic oligonucleotide
ttcatggaatgggcgagaag

SEQ ID NO: 254 - DNA, 20 bp, Artificial sequence
  Synthetic oligonucleotide
acagaggcagggcaggcacg

SEQ ID NO: 255 - DNA, 20 bp, Artificial sequence
  Synthetic oligonucleotide
aagattcatgcttgttagaa

SEQ ID NO: 256 - DNA, 20 bp, Artificial sequence
  Synthetic oligonucleotide
tcaaagcaggaactggtgag

SEQ ID NO: 257 - DNA, 20 bp, Artificial sequence
  Synthetic oligonucleotide
ggtctacagaagcaaggtgt

SEQ ID NO: 258 - DNA, 20 bp, Artificial sequence
  Synthetic oligonucleotide
catcccagctaccatggaat

SEQ ID NO: 259 - DNA, 20 bp, Artificial sequence
  Synthetic oligonucleotide
caccatcctgaggccaggca

SEQ ID NO: 260 - DNA, 20 bp, Artificial sequence
  Synthetic oligonucleotide
taacttttttctattattat

SEQ ID NO: 261 - DNA, 20 bp, Artificial sequence
  Synthetic oligonucleotide
acagtcacagaacaacaaag

SEQ ID NO: 262 - DNA, 20 bp, Artificial sequence
  Synthetic oligonucleotide
ggcctaattttttatctttg

SEQ ID NO: 263 - DNA, 20 bp, Artificial sequence
  Synthetic oligonucleotide
acagggttgtagccatcagc

SEQ ID NO: 264 - DNA, 20 bp, Artificial sequence
  Synthetic oligonucleotide
gatcactggaacacaatggt

SEQ ID NO: 265 - DNA, 20 bp, Artificial sequence
  Synthetic oligonucleotide
ggaagagaaaagaagggcac

SEQ ID NO: 266 - DNA, 20 bp, Artificial sequence
  Synthetic oligonucleotide
catttaataaataaatccct

SEQ ID NO: 267 - DNA, 20 bp, Artificial sequence
  Synthetic oligonucleotide
tttaccagtgccatttttcc

SEQ ID NO: 268 - DNA, 20 bp, Artificial sequence
  Synthetic oligonucleotide
cagcaaatttctgtggtttt

SEQ ID NO: 269 - DNA, 20 bp, Artificial sequence
  Synthetic oligonucleotide
gctctcagaccagaccagac

SEQ ID NO: 270 - DNA, 20 bp, Artificial sequence
  Synthetic oligonucleotide
acagctgatgaggagggtgg

SEQ ID NO: 271 - DNA, 20 bp, Artificial sequence
  Synthetic oligonucleotide
tacacaaatactaagccaca

SEQ ID NO: 272 - DNA, 20 bp, Artificial sequence
  Synthetic oligonucleotide
actgccaccaccatgactaa

SEQ ID NO: 273 - DNA, 20 bp, Artificial sequence
  Synthetic oligonucleotide
gttagaagttgattttttct

SEQ ID NO: 274 - DNA, 20 bp, Artificial sequence
  Synthetic oligonucleotide
atactcacatggtggagaaa

SEQ ID NO: 275 - DNA, 20 bp, Artificial sequence
  Synthetic oligonucleotide
gagaagaatggaagggagaa

SEQ ID NO: 276 - DNA, 20 bp, Artificial sequence
  Synthetic oligonucleotide
tagagggttggaggaacagg

SEQ ID NO: 277 - DNA, 20 bp, Artificial sequence
  Synthetic oligonucleotide
cttagaacaaagagaagaat

SEQ ID NO: 278 - DNA, 20 bp, Artificial sequence
  Synthetic oligonucleotide
gacactgacactgtgcatga

SEQ ID NO: 279 - DNA, 20 bp, Artificial sequence
  Synthetic oligonucleotide
ggagttaccatatgacctgg

SEQ ID NO: 280 - DNA, 20 bp, Artificial sequence
  Synthetic oligonucleotide
cgtaagcttctagcaaggag

SEQ ID NO: 281 - DNA, 20 bp, Artificial sequence
  Synthetic oligonucleotide
ggtaaaaatgataaaaaacg

SEQ ID NO: 282 - DNA, 20 bp, Artificial sequence
  Synthetic oligonucleotide
agccttctcctgcctcagct

SEQ ID NO: 283 - DNA, 20 bp, Artificial sequence
  Synthetic oligonucleotide
agaagcagcagccacctgcg

SEQ ID NO: 284 - DNA, 20 bp, Artificial sequence
  Synthetic oligonucleotide
tggtcttctgacttttcttc

SEQ ID NO: 285 - DNA, 20 bp, Artificial sequence
  Synthetic oligonucleotide
cacctttttaaacttgaggg

SEQ ID NO: 286 - DNA, 20 bp, Artificial sequence
  Synthetic oligonucleotide
tttctcttctttcttatctt

SEQ ID NO: 287 - DNA, 20 bp, Artificial sequence
  Synthetic oligonucleotide
tcatgcttgccctctttctc

SEQ ID NO: 288 - DNA, 20 bp, Artificial sequence
  Synthetic oligonucleotide
tgatggctgcacgggctcat

SEQ ID NO: 289 - DNA, 20 bp, Artificial sequence
  Synthetic oligonucleotide
cagcagagtggtgggctgat

SEQ ID NO: 290 - DNA, 20 bp, Artificial sequence
  Synthetic oligonucleotide
tgatgtctctgctttgcctg

SEQ ID NO: 291 - DNA, 20 bp, Artificial sequence
  Synthetic oligonucleotide
cagaagcttccggcacagcc

SEQ ID NO: 292 - DNA, 20 bp, Artificial sequence
  Synthetic oligonucleotide
gggtccccggtcacggatga

SEQ ID NO: 293 - DNA, 20 bp, Artificial sequence
  Synthetic oligonucleotide
gcttaagcttccgtgtccag

SEQ ID NO: 294 - DNA, 20 bp, Artificial sequence
  Synthetic oligonucleotide
atacttcccagcagagcggc

SEQ ID NO: 295 - DNA, 20 bp, Artificial sequence
  Synthetic oligonucleotide
agcaaccaaagagtcaggcc

SEQ ID NO: 296 - DNA, 20 bp, Artificial sequence
  Synthetic oligonucleotide
actttagagcgaaaggcttt

SEQ ID NO: 297 - DNA, 20 bp, Artificial sequence
  Synthetic oligonucleotide
ttttcgaagtacgcaatcaa

SEQ ID NO: 298 - DNA, 20 bp, Artificial sequence
  Synthetic oligonucleotide
ccagggatgtgtcgcctacc

SEQ ID NO: 299 - DNA, 20 bp, Artificial sequence
  Synthetic oligonucleotide
ccagttaccgtgaagtcaaa

SEQ ID NO: 300 - DNA, 20 bp, Artificial sequence
  Synthetic oligonucleotide
tgggcttcttaggtggtttc

SEQ ID NO: 301 - DNA, 20 bp, Artificial sequence
  Synthetic oligonucleotide
gtggtgccgctccctttggg

SEQ ID NO: 302 - DNA, 20 bp, Artificial sequence
  Synthetic oligonucleotide
tctccaggacccttttcacc

SEQ ID NO: 303 - DNA, 20 bp, Artificial sequence
  Synthetic oligonucleotide
gacaaggagcttcccaggac

SEQ ID NO: 304 - DNA, 20 bp, Artificial sequence
  Synthetic oligonucleotide
ccctggcgaagtttgaaaag

SEQ ID NO: 305 - DNA, 20 bp, Artificial sequence
  Synthetic oligonucleotide
cccctcagccttgccccctg

SEQ ID NO: 306 - DNA, 20 bp, Artificial sequence
  Synthetic oligonucleotide
tgggtggatgtggtggcccc

SEQ ID NO: 307 - DNA, 20 bp, Artificial sequence
  Synthetic oligonucleotide
cggcctcagcttttcgcttc

SEQ ID NO: 308 - DNA, 20 bp, Artificial sequence
  Synthetic oligonucleotide
tcggccccgtttcttgggaa

SEQ ID NO: 309 - DNA, 20 bp, Artificial sequence
  Synthetic oligonucleotide
gcggcagcggctgccaccac

SEQ ID NO: 310 - DNA, 20 bp, Artificial sequence
  Synthetic oligonucleotide
aagactccttcacggctttc

SEQ ID NO: 311 - DNA, 20 bp, Artificial sequence
  Synthetic oligonucleotide
ggtctcctgcacagatcgga

SEQ ID NO: 312 - DNA, 20 bp, Artificial sequence
  Synthetic oligonucleotide
gctgaccgtctcccgggtct

SEQ ID NO: 313 - DNA, 20 bp, Artificial sequence
  Synthetic oligonucleotide
cgagggtggacaccagcagg

SEQ ID NO: 314 - DNA, 20 bp, Artificial sequence
  Synthetic oligonucleotide
acaggtcttcagtcctttcc

SEQ ID NO: 315 - DNA, 20 bp, Artificial sequence
  Synthetic oligonucleotide
ctgctctccttgcttttccg

SEQ ID NO: 316 - DNA, 20 bp, Artificial sequence
  Synthetic oligonucleotide
ctgagtggtggtgatggtgg

SEQ ID NO: 317 - DNA, 20 bp, Artificial sequence
  Synthetic oligonucleotide
cttctcctctttgcagacgc

SEQ ID NO: 318 - DNA, 20 bp, Artificial sequence
  Synthetic oligonucleotide
ccgtcgctctccagtgagcc

SEQ ID NO: 319 - DNA, 20 bp, Artificial sequence
  Synthetic oligonucleotide
ggcaaccgcgggctgagtct

SEQ ID NO: 320 - DNA, 20 bp, Artificial sequence
  Synthetic oligonucleotide
ccgtggcggcggtggcaacc

SEQ ID NO: 321 - DNA, 20 bp, Artificial sequence
  Synthetic oligonucleotide
tacttttctgcggccgtggc

SEQ ID NO: 322 - DNA, 20 bp, Artificial sequence
  Synthetic oligonucleotide
tctttgcgctctccctcccc

SEQ ID NO: 323 - DNA, 20 bp, Artificial sequence
  Synthetic oligonucleotide
tgtttggccttggcatggag

SEQ ID NO: 324 - DNA, 20 bp, Artificial sequence
  Synthetic oligonucleotide
aactctctcggtcacgggcg

SEQ ID NO: 325 - DNA, 20 bp, Artificial sequence
  Synthetic oligonucleotide
tgctttgcaatccgctccgt

SEQ ID NO: 326 - DNA, 20 bp, Artificial sequence
  Synthetic oligonucleotide
agagacaacagctgccttta

SEQ ID NO: 327 - DNA, 20 bp, Artificial sequence
  Synthetic oligonucleotide
gaagctttgtcagagcccta

SEQ ID NO: 328 - DNA, 22 bp, Artificial sequence
  Synthetic oligonucleotide
ccttccctgaaggttccctccc